European Patent Application EP 4 537 904 A2, published April 16, 2025. Title: MULTI-SPECIFIC BINDING PROTEINS AND IMPROVEMENTS THEREON. Applicant: DRAGONFLY THERAPEUTICS, INC. Application EP. The sequence listing filed with the application follows.

SEQUENCE LISTING (445 sequences)

SEQ ID NO: 1 - protein, 117 aa, synthetic construct
  REGION 1..117: note = Description of Artificial Sequence: Synthetic polypeptide
QVQLQQWGAGLLKPSETLSLTCAVYGGSFSGYYWSWIRQPPGKGLEWIGEIDHSGSTNYNPSLKSRVTISVDTSKNQFSLKLSSVTAADTAVYYCARARGPWSFDPWGQGTLVTVSS

SEQ ID NO: 2 - protein, 107 aa, synthetic construct
  REGION 1..107: note = Description of Artificial Sequence: Synthetic polypeptide
DIQMTQSPSTLSASVGDRVTITCRASQSISSWLAWYQQKPGKAPKLLIYKASSLESGVPSRFSGSGSGTEFTLTISSLQPDDFATYYCQQYNSYPITFGGGTKVEIK

SEQ ID NO: 3 - protein, 9 aa, synthetic construct
  REGION 1..9: note = Description of Artificial Sequence: Synthetic peptide
GSFSGYYWS

SEQ ID NO: 4 - protein, 16 aa, synthetic construct
  REGION 1..16: note = Description of Artificial Sequence: Synthetic peptide
EIDHSGSTNYNPSLKS

SEQ ID NO: 5 - protein, 11 aa, synthetic construct
  REGION 1..11: note = Description of Artificial Sequence: Synthetic peptide
ARARGPWSFDP

SEQ ID NO: 6 - protein, 117 aa, synthetic construct; identical to SEQ ID NO: 1
  REGION 1..117: note = Description of Artificial Sequence: Synthetic polypeptide

SEQ ID NO: 7 - protein, 108 aa, synthetic construct
  REGION 1..108: note = Description of Artificial Sequence: Synthetic polypeptide
EIVLTQSPGTLSLSPGERATLSCRASQSVSSSYLAWYQQKPGQAPRLLIYGASSRATGIPDRFSGSGSGTDFTLTISRLEPEDFAVYYCQQYGSSPITFGGGTKVEIK

SEQ ID NO: 8 - protein, 117 aa, synthetic construct; identical to SEQ ID NO: 1
  REGION 1..117: note = Description of Artificial Sequence: Synthetic polypeptide

SEQ ID NO: 9 - protein, 106 aa, synthetic construct
  REGION 1..106: note = Description of Artificial Sequence: Synthetic polypeptide
DIQMTQSPSTLSASVGDRVTITCRASQSIGSWLAWYQQKPGKAPKLLIYKASSLESGVPSRFSGSGSGTEFTLTISSLQPDDFATYYCQQYHSFYTFGGGTKVEIK

SEQ ID NO: 10 - protein, 117 aa, synthetic construct; identical to SEQ ID NO: 1
  REGION 1..117: note = Description of Artificial Sequence: Synthetic polypeptide

SEQ ID NO: 11 - protein, 106 aa, synthetic construct
  REGION 1..106: note = Description of Artificial Sequence: Synthetic polypeptide
DIQMTQSPSTLSASVGDRVTITCRASQSIGSWLAWYQQKPGKAPKLLIYKASSLESGVPSRFSGSGSGTEFTLTISSLQPDDFATYYCQQSNSYYTFGGGTKVEIK

SEQ ID NO: 12 - protein, 117 aa, synthetic construct; identical to SEQ ID NO: 1
  REGION 1..117: note = Description of Artificial Sequence: Synthetic polypeptide

SEQ ID NO: 13 - protein, 106 aa, synthetic construct
  REGION 1..106: note = Description of Artificial Sequence: Synthetic polypeptide
DIQMTQSPSTLSASVGDRVTITCRASQSISSWLAWYQQKPGKAPKLLIYKASSLESGVPSRFSGSGSGTEFTLTISSLQPDDFATYYCQQYNSYPTFGGGTKVEIK

SEQ ID NO: 14 - protein, 117 aa, synthetic construct
  REGION 1..117: note = Description of Artificial Sequence: Synthetic polypeptide
QVQLQQWGAGLLKPSETLSLTCAVYGGSFSGYYWSWIRQPPGKGLEWIGEIDHSGSTNYNPSLKSRVTISVDTSKNQFSLKLSSVTAADTAVYYCARARGPWGFDPWGQGTLVTVSS

SEQ ID NO: 15 - protein, 107 aa, synthetic construct
  REGION 1..107: note = Description of Artificial Sequence: Synthetic polypeptide
ELQMTQSPSSLSASVGDRVTITCRTSQSISSYLNWYQQKPGQPPKLLIYWASTRESGVPDRFSGSGSGTDFTLTISSLQPEDSATYYCQQSYDIPYTFGQGTKLEIK

SEQ ID NO: 16 - protein, 117 aa, synthetic construct; identical to SEQ ID NO: 1
  REGION 1..117: note = Description of Artificial Sequence: Synthetic polypeptide

SEQ ID NO: 17 - protein, 107 aa, synthetic construct
  REGION 1..107: note = Description of Artificial Sequence: Synthetic polypeptide
DIQMTQSPSTLSASVGDRVTITCRASQSISSWLAWYQQKPGKAPKLLIYKASSLESGVPSRFSGSGSGTEFTLTISSLQPDDFATYYCQQYGSFPITFGGGTKVEIK

SEQ ID NO: 18 - protein, 117 aa, synthetic construct; identical to SEQ ID NO: 1
  REGION 1..117: note = Description of Artificial Sequence: Synthetic polypeptide

SEQ ID NO: 19 - protein, 107 aa, synthetic construct
  REGION 1..107: note = Description of Artificial Sequence: Synthetic polypeptide
DIQMTQSPSTLSASVGDRVTITCRASQSISSWLAWYQQKPGKAPKLLIYKASSLESGVPSRFSGSGSGTDFTLTISSLQPDDFATYYCQQSKEVPWTFGQGTKVEIK

SEQ ID NO: 20 - protein, 117 aa, synthetic construct; identical to SEQ ID NO: 1
  REGION 1..117: note = Description of Artificial Sequence: Synthetic polypeptide

SEQ ID NO: 21 - protein, 106 aa, synthetic construct
  REGION 1..106: note = Description of Artificial Sequence: Synthetic polypeptide
DIQMTQSPSTLSASVGDRVTITCRASQSISSWLAWYQQKPGKAPKLLIYKASSLESGVPSRFSGSGSGTEFTLTISSLQPDDFATYYCQQYNSFPTFGGGTKVEIK

SEQ ID NO: 22 - protein, 117 aa, synthetic construct; identical to SEQ ID NO: 1
  REGION 1..117: note = Description of Artificial Sequence: Synthetic polypeptide

SEQ ID NO: 23 - protein, 106 aa, synthetic construct
  REGION 1..106: note = Description of Artificial Sequence: Synthetic polypeptide
DIQMTQSPSTLSASVGDRVTITCRASQSIGSWLAWYQQKPGKAPKLLIYKASSLESGVPSRFSGSGSGTEFTLTISSLQPDDFATYYCQQYDIYPTFGGGTKVEIK

SEQ ID NO: 24 - protein, 117 aa, synthetic construct; identical to SEQ ID NO: 1
  REGION 1..117: note = Description of Artificial Sequence: Synthetic polypeptide

SEQ ID NO: 25 - protein, 106 aa, synthetic construct
  REGION 1..106: note = Description of Artificial Sequence: Synthetic polypeptide
DIQMTQSPSTLSASVGDRVTITCRASQSISSWLAWYQQKPGKAPKLLIYKASSLESGVPSRFSGSGSGTEFTLTISSLQPDDFATYYCQQYDSYPTFGGGTKVEIK

SEQ ID NO: 26 - protein, 117 aa, synthetic construct; identical to SEQ ID NO: 1
  REGION 1..117: note = Description of Artificial Sequence: Synthetic polypeptide

SEQ ID NO: 27 - protein, 106 aa, synthetic construct
  REGION 1..106: note = Description of Artificial Sequence: Synthetic polypeptide
DIQMTQSPSTLSASVGDRVTITCRASQSISSWLAWYQQKPGKAPKLLIYKASSLESGVPSRFSGSGSGTEFTLTISSLQPDDFATYYCQQYGSFPTFGGGTKVEIK

SEQ ID NO: 28 - protein, 117 aa, synthetic construct; identical to SEQ ID NO: 1
  REGION 1..117: note = Description of Artificial Sequence: Synthetic polypeptide

SEQ ID NO: 29 - protein, 106 aa, synthetic construct
  REGION 1..106: note = Description of Artificial Sequence: Synthetic polypeptide
DIQMTQSPSTLSASVGDRVTITCRASQSISSWLAWYQQKPGKAPKLLIYKASSLESGVPSRFSGSGSGTEFTLTISSLQPDDFATYYCQQYQSFPTFGGGTKVEIK

SEQ ID NO: 30 - protein, 117 aa, synthetic construct; identical to SEQ ID NO: 1
  REGION 1..117: note = Description of Artificial Sequence: Synthetic polypeptide

SEQ ID NO: 31 - protein, 106 aa, synthetic construct
  REGION 1..106: note = Description of Artificial Sequence: Synthetic polypeptide
DIQMTQSPSTLSASVGDRVTITCRASQSISSWLAWYQQKPGKAPKLLIYKASSLESGVPSRFSGSGSGTEFTLTISSLQPDDFATYYCQQYSSFSTFGGGTKVEIK

SEQ ID NO: 32 - protein, 117 aa, synthetic construct; identical to SEQ ID NO: 1
  REGION 1..117: note = Description of Artificial Sequence: Synthetic polypeptide

SEQ ID NO: 33 - protein, 106 aa, synthetic construct
  REGION 1..106: note = Description of Artificial Sequence: Synthetic polypeptide
DIQMTQSPSTLSASVGDRVTITCRASQSISSWLAWYQQKPGKAPKLLIYKASSLESGVPSRFSGSGSGTEFTLTISSLQPDDFATYYCQQYESYSTFGGGTKVEIK

SEQ ID NO: 34 - protein, 117 aa, synthetic construct; identical to SEQ ID NO: 1
  REGION 1..117: note = Description of Artificial Sequence: Synthetic polypeptide

SEQ ID NO: 35 - protein, 106 aa, synthetic construct
  REGION 1..106: note = Description of Artificial Sequence: Synthetic polypeptide
DIQMTQSPSTLSASVGDRVTITCRASQSISSWLAWYQQKPGKAPKLLIYKASSLESGVPSRFSGSGSGTEFTLTISSLQPDDFATYYCQQYDSFITFGGGTKVEIK

SEQ ID NO: 36 - protein, 117 aa, synthetic construct; identical to SEQ ID NO: 1
  REGION 1..117: note = Description of Artificial Sequence: Synthetic polypeptide

SEQ ID NO: 37 - protein, 106 aa, synthetic construct
  REGION 1..106: note = Description of Artificial Sequence: Synthetic polypeptide
DIQMTQSPSTLSASVGDRVTITCRASQSISSWLAWYQQKPGKAPKLLIYKASSLESGVPSRFSGSGSGTEFTLTISSLQPDDFATYYCQQYQSYPTFGGGTKVEIK

SEQ ID NO: 38 - protein, 117 aa, synthetic construct; identical to SEQ ID NO: 1
  REGION 1..117: note = Description of Artificial Sequence: Synthetic polypeptide

SEQ ID NO: 39 - protein, 106 aa, synthetic construct
  REGION 1..106: note = Description of Artificial Sequence: Synthetic polypeptide
DIQMTQSPSTLSASVGDRVTITCRASQSIGSWLAWYQQKPGKAPKLLIYKASSLESGVPSRFSGSGSGTEFTLTISSLQPDDFATYYCQQYHSFPTFGGGTKVEIK

SEQ ID NO: 40 - protein, 117 aa, synthetic construct; identical to SEQ ID NO: 1
  REGION 1..117: note = Description of Artificial Sequence: Synthetic polypeptide

SEQ ID NO: 41 - protein, 107 aa, synthetic construct
  REGION 1..107: note = Description of Artificial Sequence: Synthetic polypeptide
DIQMTQSPSTLSASVGDRVTITCRASQSIGSWLAWYQQKPGKAPKLLIYKASSLESGVPSRFSGSGSGTEFTLTISSLQPDDFATYYCQQYELYSYTFGGGTKVEIK

SEQ ID NO: 42 - protein, 117 aa, synthetic construct; identical to SEQ ID NO: 1
  REGION 1..117: note = Description of Artificial Sequence: Synthetic polypeptide

SEQ ID NO: 43 - protein, 106 aa, synthetic construct
  REGION 1..106: note = Description of Artificial Sequence: Synthetic polypeptide
DIQMTQSPSTLSASVGDRVTITCRASQSISSWLAWYQQKPGKAPKLLIYKASSLESGVPSRFSGSGSGTEFTLTISSLQPDDFATYYCQQYDTFITFGGGTKVEIK

SEQ ID NO: 44 - protein, 125 aa, synthetic construct
  REGION 1..125: note = Description of Artificial Sequence: Synthetic polypeptide
QVQLVQSGAEVKKPGSSVKVSCKASGGTFSSYAISWVRQAPGQGLEWMGGIIPIFGTANYAQKFQGRVTITADESTSTAYMELSSLRSEDTAVYYCARGDSSIRHAYYYYGMDVWGQGTTVTVSS

SEQ ID NO: 45 - protein, 9 aa, synthetic construct
  REGION 1..9: note = Description of Artificial Sequence: Synthetic peptide
GTFSSYAIS

SEQ ID NO: 46 - protein, 17 aa, synthetic construct
  REGION 1..17: note = Description of Artificial Sequence: Synthetic peptide
GIIPIFGTANYAQKFQG

SEQ ID NO: 47 - protein, 18 aa, synthetic construct
  REGION 1..18: note = Description of Artificial Sequence: Synthetic peptide
ARGDSSIRHAYYYYGMDV

SEQ ID NO: 48 - protein, 113 aa, synthetic construct
  REGION 1..113: note = Description of Artificial Sequence: Synthetic polypeptide
DIVMTQSPDSLAVSLGERATINCKSSQSVLYSSNNKNYLAWYQQKPGQPPKLLIYWASTRESGVPDRFSGSGSGTDFTLTISSLQAEDVAVYYCQQYYSTPITFGGGTKVEIK

SEQ ID NO: 49 - protein, 17 aa, synthetic construct
  REGION 1..17: note = Description of Artificial Sequence: Synthetic peptide
KSSQSVLYSSNNKNYLA

SEQ ID NO: 50 - protein, 7 aa, synthetic construct
  REGION 1..7: note = Description of Artificial Sequence: Synthetic peptide
WASTRES

SEQ ID NO: 51 - protein, 9 aa, synthetic construct
  REGION 1..9: note = Description of Artificial Sequence: Synthetic peptide
QQYYSTPIT

SEQ ID NO: 52 - protein, 121 aa, synthetic construct
  REGION 1..121: note = Description of Artificial Sequence: Synthetic polypeptide
QLQLQESGPGLVKPSETLSLTCTVSGGSISSSSYYWGWIRQPPGKGLEWIGSIYYSGSTYYNPSLKSRVTISVDTSKNQFSLKLSSVTAADTAVYYCARGSDRFHPYFDYWGQGTLVTVSS

SEQ ID NO: 53 - protein, 11 aa, synthetic construct
  REGION 1..11: note = Description of Artificial Sequence: Synthetic peptide
GSISSSSYYWG

SEQ ID NO: 54 - protein, 16 aa, synthetic construct
  REGION 1..16: note = Description of Artificial Sequence: Synthetic peptide
SIYYSGSTYYNPSLKS

SEQ ID NO: 55 - protein, 13 aa, synthetic construct
  REGION 1..13: note = Description of Artificial Sequence: Synthetic peptide
ARGSDRFHPYFDY

SEQ ID NO: 56 - protein, 107 aa, synthetic construct
  REGION 1..107: note = Description of Artificial Sequence: Synthetic polypeptide
EIVLTQSPATLSLSPGERATLSCRASQSVSRYLAWYQQKPGQAPRLLIYDASNRATGIPARFSGSGSGTDFTLTISSLEPEDFAVYYCQQFDTWPPTFGGGTKVEIK

SEQ ID NO: 57 - protein, 11 aa, synthetic construct
  REGION 1..11: note = Description of Artificial Sequence: Synthetic peptide
RASQSVSRYLA

SEQ ID NO: 58 - protein, 7 aa, synthetic construct
  REGION 1..7: note = Description of Artificial Sequence: Synthetic peptide
DASNRAT

SEQ ID NO: 59 - protein, 9 aa, synthetic construct
  REGION 1..9: note = Description of Artificial Sequence: Synthetic peptide
QQFDTWPPT

SEQ ID NO: 60 - protein, 117 aa, synthetic construct; identical to SEQ ID NO: 1
  REGION 1..117: note = Description of Artificial Sequence: Synthetic polypeptide

SEQ ID NO: 61 - protein, 106 aa, synthetic construct
  REGION 1..106: note = Description of Artificial Sequence: Synthetic polypeptide
DIQMTQSPSTLSASVGDRVTITCRASQSISSWLAWYQQKPGKAPKLLIYKASSLESGVPSRFSGSGSGTEFTLTISSLQPDDFATYYCEQYDSYPTFGGGTKVEIK

SEQ ID NO: 62 - protein, 126 aa, synthetic construct
  REGION 1..126: note = Description of Artificial Sequence: Synthetic polypeptide
QVQLVQSGAEVKKPGSSVKVSCKASGGTFSSYAISWVRQAPGQGLEWMGGIIPIFGTANYAQKFQGRVTITADESTSTAYMELSSLRSEDTAVYYCARRGRKASGSFYYYYGMDVWGQGTTVTVSS

SEQ ID NO: 63 - protein, 9 aa, synthetic construct
  REGION 1..9: note = Description of Artificial Sequence: Synthetic peptide
GTFSSYAIS

SEQ ID NO: 64 - protein, 17 aa, synthetic construct
  REGION 1..17: note = Description of Artificial Sequence: Synthetic peptide
GIIPIFGTANYAQKFQG

SEQ ID NO: 65 - protein, 19 aa, synthetic construct
  REGION 1..19: note = Description of Artificial Sequence: Synthetic peptide
ARRGRKASGSFYYYYGMDV

SEQ ID NO: 66 - protein, 113 aa, synthetic construct [sequence omitted]

SEQ ID NO: 67 - protein, 17 aa, synthetic construct
  REGION 1..17: note = Description of Artificial Sequence: Synthetic peptide
ESSQSLLNSGNQKNYLT

SEQ ID NO: 68 - protein, 7 aa, synthetic construct
  REGION 1..7: note = Description of Artificial Sequence: Synthetic peptide
WASTRES

SEQ ID NO: 69 - protein, 9 aa, synthetic construct
  REGION 1..9: note = Description of Artificial Sequence: Synthetic peptide
QNDYSYPYT

SEQ ID NO: 70 - protein, 126 aa, synthetic construct
  REGION 1..126: note = Description of Artificial Sequence: Synthetic polypeptide
QVQLVQSGAEVKKPGASVKVSCKASGYTFTSYYMHWVRQAPGQGLEWMGIINPSGGSTSYAQKFQGRVTMTRDTSTSTVYMELSSLRSEDTAVYYCARGAPNYGDTTHDYYYMDVWGKGTTVTVSS

SEQ ID NO: 71 - protein, 9 aa, synthetic construct
  REGION 1..9: note = Description of Artificial Sequence: Synthetic peptide
YTFTSYYMH

SEQ ID NO: 72 - protein, 17 aa, synthetic construct
  REGION 1..17: note = Description of Artificial Sequence: Synthetic peptide
IINPSGGSTSYAQKFQG

SEQ ID NO: 73 - protein, 19 aa, synthetic construct
  REGION 1..19: note = Description of Artificial Sequence: Synthetic peptide
ARGAPNYGDTTHDYYYMDV

SEQ ID NO: 74 - protein, 107 aa, synthetic construct
  REGION 1..107: note = Description of Artificial Sequence: Synthetic polypeptide
EIVMTQSPATLSVSPGERATLSCRASQSVSSNLAWYQQKPGQAPRLLIYGASTRATGIPARFSGSGSGTEFTLTISSLQSEDFAVYYCQQYDDWPFTFGGGTKVEIK

SEQ ID NO: 75 - protein, 11 aa, synthetic construct
  REGION 1..11: note = Description of Artificial Sequence: Synthetic peptide
RASQSVSSNLA

SEQ ID NO: 76 - protein, 7 aa, synthetic construct
  REGION 1..7: note = Description of Artificial Sequence: Synthetic peptide
GASTRAT

SEQ ID NO: 77 - protein, 9 aa, synthetic construct
  REGION 1..9: note = Description of Artificial Sequence: Synthetic peptide
QQYDDWPFT

SEQ ID NO: 78 - protein, 124 aa, synthetic construct
  REGION 1..124: note = Description of Artificial Sequence: Synthetic polypeptide
QVQLVQSGAEVKKPGASVKVSCKASGYTFTGYYMHWVRQAPGQGLEWMGWINPNSGGTNYAQKFQGRVTMTRDTSISTAYMELSRLRSDDTAVYYCARDTGEYYDTDDHGMDVWGQGTTVTVSS

SEQ ID NO: 79 - protein, 9 aa, synthetic construct
  REGION 1..9: note = Description of Artificial Sequence: Synthetic peptide
YTFTGYYMH

SEQ ID NO: 80 - protein, 17 aa, synthetic construct
  REGION 1..17: note = Description of Artificial Sequence: Synthetic peptide
WINPNSGGTNYAQKFQG

SEQ ID NO: 81 - protein, 17 aa, synthetic construct
  REGION 1..17: note = Description of Artificial Sequence: Synthetic peptide
ARDTGEYYDTDDHGMDV

SEQ ID NO: 82 - protein, 107 aa, synthetic construct
  REGION 1..107: note = Description of Artificial Sequence: Synthetic polypeptide
EIVLTQSPGTLSLSPGERATLSCRASQSVSSNLAWYQQKPGQAPRLLIYGASTRATGIPARFSGSGSGTEFTLTISSLQSEDFAVYYCQQDDYWPPTFGGGTKVEIK

SEQ ID NO: 83 - protein, 11 aa, synthetic construct
  REGION 1..11: note = Description of Artificial Sequence: Synthetic peptide
RASQSVSSNLA

SEQ ID NO: 84 - protein, 7 aa, synthetic construct
  REGION 1..7: note = Description of Artificial Sequence: Synthetic peptide
GASTRAT

SEQ ID NO: 85 - protein, 9 aa, synthetic construct
  REGION 1..9: note = Description of Artificial Sequence: Synthetic peptide
QQDDYWPPT

SEQ ID NO: 86 - protein, 121 aa, synthetic construct
  REGION 1..121: note = Description of Artificial Sequence: Synthetic polypeptide
EVQLLESGGGLVQPGGSLRLSCAASGFTFSSYAMSWVRQAPGKGLEWVSAISGSGGSTYYADSVKGRFTISRDNSKNTLYLQMNSLRAEDTAVYYCAKDGGYYDSGAGDYWGQGTLVTVSS

SEQ ID NO: 87 - protein, 9 aa, synthetic construct
  REGION 1..9: note = Description of Artificial Sequence: Synthetic peptide
FTFSSYAMS

SEQ ID NO: 88 - protein, 17 aa, synthetic construct
  REGION 1..17: note = Description of Artificial Sequence: Synthetic peptide
AISGSGGSTYYADSVKG

SEQ ID NO: 89 - protein, 14 aa, synthetic construct
  REGION 1..14: note = Description of Artificial Sequence: Synthetic peptide
AKDGGYYDSGAGDY

SEQ ID NO: 90 - protein, 107 aa, synthetic construct
  REGION 1..107: note = Description of Artificial Sequence: Synthetic polypeptide
DIQMTQSPSSVSASVGDRVTITCRASQGIDSWLAWYQQKPGKAPKLLIYAASSLQSGVPSRFSGSGSGTDFTLTISSLQPEDFATYYCQQGVSYPRTFGGGTKVEIK

SEQ ID NO: 91 - protein, 11 aa, synthetic construct
  REGION 1..11: note = Description of Artificial Sequence: Synthetic peptide
RASQGIDSWLA

SEQ ID NO: 92 - protein, 7 aa, synthetic construct
  REGION 1..7: note = Description of Artificial Sequence: Synthetic peptide
AASSLQS

SEQ ID NO: 93 - protein, 9 aa, synthetic construct
  REGION 1..9: note = Description of Artificial Sequence: Synthetic peptide
QQGVSYPRT

SEQ ID NO: 94 - protein, 122 aa, synthetic construct
  REGION 1..122: note = Description of Artificial Sequence: Synthetic polypeptide
EVQLVESGGGLVKPGGSLRLSCAASGFTFSSYSMNWVRQAPGKGLEWVSSISSSSSYIYYADSVKGRFTISRDNAKNSLYLQMNSLRAEDTAVYYCARGAPMGAAAGWFDPWGQGTLVTVSS

SEQ ID NO: 95 - protein, 9 aa, synthetic construct
  REGION 1..9: note = Description of Artificial Sequence: Synthetic peptide
FTFSSYSMN

SEQ ID NO: 96 - protein, 17 aa, synthetic construct
  REGION 1..17: note = Description of Artificial Sequence: Synthetic peptide
SISSSSSYIYYADSVKG

SEQ ID NO: 97 - protein, 15 aa, synthetic construct
  REGION 1..15: note = Description of Artificial Sequence: Synthetic peptide
ARGAPMGAAAGWFDP

SEQ ID NO: 98 - protein, 107 aa, synthetic construct
  REGION 1..107: note = Description of Artificial Sequence: Synthetic polypeptide
DIQMTQSPSSVSASVGDRVTITCRASQGISSWLAWYQQKPGKAPKLLIYAASSLQSGVPSRFSGSGSGTDFTLTISSLQPEDFATYYCQQGVSFPRTFGGGTKVEIK

SEQ ID NO: 99 - protein, 11 aa, synthetic construct
  REGION 1..11: note = Description of Artificial Sequence: Synthetic peptide
RASQGISSWLA

SEQ ID NO: 100 - protein, 7 aa, synthetic construct
  REGION 1..7: note = Description of Artificial Sequence: Synthetic peptide
AASSLQS

SEQ ID NO: 101 - protein, 9 aa, synthetic construct
  REGION 1..9: note = Description of Artificial Sequence: Synthetic peptide
QQGVSFPRT

SEQ ID NO: 102 - protein, 125 aa, synthetic construct
  REGION 1..125: note = Description of Artificial Sequence: Synthetic polypeptide
QVQLVQSGAEVKKPGASVKVSCKASGYTFTSYYMHWVRQAPGQGLEWMGIINPSGGSTSYAQKFQGRVTMTRDTSTSTVYMELSSLRSEDTAVYYCAREGAGFAYGMDYYYMDVWGKGTTVTVSS

SEQ ID NO: 103 - protein, 9 aa, synthetic construct
  REGION 1..9: note = Description of Artificial Sequence: Synthetic peptide
YTFTSYYMH

SEQ ID NO: 104 - protein, 17 aa, synthetic construct
  REGION 1..17: note = Description of Artificial Sequence: Synthetic peptide
IINPSGGSTSYAQKFQG

SEQ ID NO: 105 - protein, 18 aa, synthetic construct
  REGION 1..18: note = Description of Artificial Sequence: Synthetic peptide
AREGAGFAYGMDYYYMDV

SEQ ID NO: 106 - protein, 107 aa, synthetic construct
  REGION 1..107: note = Description of Artificial Sequence: Synthetic polypeptide
EIVLTQSPATLSLSPGERATLSCRASQSVSSYLAWYQQKPGQAPRLLIYDASNRATGIPARFSGSGSGTDFTLTISSLEPEDFAVYYCQQSDNWPFTFGGGTKVEIK

SEQ ID NO: 107 - protein, 11 aa, synthetic construct
  REGION 1..11: note = Description of Artificial Sequence: Synthetic peptide
RASQSVSSYLA

SEQ ID NO: 108 - protein, 7 aa, synthetic construct
  REGION 1..7: note = Description of Artificial Sequence: Synthetic peptide
DASNRAT

SEQ ID NO: 109 - protein, 9 aa, synthetic construct
  REGION 1..9: note = Description of Artificial Sequence: Synthetic peptide
QQSDNWPFT

SEQ ID NO: 110 - protein, 121 aa, synthetic construct
  REGION 1..121: note = Description of Artificial Sequence: Synthetic polypeptide
QVQLVESGGGLVKPGGSLRLSCAASGFTFSSYGMHWVRQAPGKGLEWVAFIRYDGSNKYYADSVKGRFTISRDNSKNTLYLQMNSLRAEDTAVYYCAKDRGLGDGTYFDYWGQGTTVTVSS

SEQ ID NO: 111 - protein, 110 aa, synthetic construct
  REGION 1..110: note = Description of Artificial Sequence: Synthetic polypeptide
QSALTQPASVSGSPGQSITISCSGSSSNIGNNAVNWYQQLPGKAPKLLIYYDDLLPSGVSDRFSGSKSGTSAFLAISGLQSEDEADYYCAAWDDSLNGPVFGGGTKLTVL

SEQ ID NO: 112 - protein, 115 aa, synthetic construct
  REGION 1..115: note = Description of Artificial Sequence: Synthetic polypeptide
QVHLQESGPGLVKPSETLSLTCTVSDDSISSYYWSWIRQPPGKGLEWIGHISYSGSANYNPSLKSRVTISVDTSKNQFSLKLSSVTAADTAVYYCANWDDAFNIWGQGTMVTVSS

SEQ ID NO: 113 - protein, 108 aa, synthetic construct
  REGION 1..108: note = Description of Artificial Sequence: Synthetic polypeptide
EIVLTQSPGTLSLSPGERATLSCRASQSVSSSYLAWYQQKPGQAPRLLIYGASSRATGIPDRFSGSGSGTDFTLTISRLEPEDFAVYYCQQYGSSPWTFGQGTKVEIK

SEQ ID NO: 114 - protein, 119 aa, synthetic construct
  REGION 1..119: note = Description of Artificial Sequence: Synthetic polypeptide
QVQLVQSGAEVKKPGASVKVSCKASGYSFPDYYINWVRQAPGQGLEWMGWIYFASGNSEYNQKFTGRVTMTRDTSSSTAYMELSSLRSEDTAVYFCASLYDYDWYFDVWGQGTMVTVSS

SEQ ID NO: 115 - protein, 5 aa, synthetic construct
  REGION 1..5: note = Description of Artificial Sequence: Synthetic peptide
DYYIN

SEQ ID NO: 116 - protein, 17 aa, synthetic construct
  REGION 1..17: note = Description of Artificial Sequence: Synthetic peptide
WIYFASGNSEYNQKFTG

SEQ ID NO: 117 - protein, 10 aa, synthetic construct
  REGION 1..10: note = Description of Artificial Sequence: Synthetic peptide
LYDYDWYFDV

SEQ ID NO: 118 - protein, 112 aa, synthetic construct
  REGION 1..112: note = Description of Artificial Sequence: Synthetic polypeptide
DIVMTQTPLSLSVTPGEPASISCKSSQSLVHSNGNTYLHWYLQKPGQSPQLLIYKVSNRFSGVPDRFSGSGSGADFTLKISRVEAEDVGVYYCAETSHVPWTFGQGTKLEIK

SEQ ID NO: 119 - protein, 112 aa, synthetic construct
  REGION 1..112: note = Description of Artificial Sequence: Synthetic polypeptide
DIVMTQTPLSLSVTPGQPASISCKSSQSLVHSNGNTYLHWYLQKPGQSPQLLIYKVSNRFSGVPDRFSGSGSGTDFTLKISRVEAEDVGIYYCSQSSIYPWTFGQGTKLEIK

SEQ ID NO: 120 - protein, 16 aa, synthetic construct
  REGION 1..16: note = Description of Artificial Sequence: Synthetic peptide
KSSQSLVHSNGNTYLH

SEQ ID NO: 121 - protein, 7 aa, synthetic construct
  REGION 1..7: note = Description of Artificial Sequence: Synthetic peptide
KVSNRFS

SEQ ID NO: 122 - protein, 9 aa, synthetic construct
  REGION 1..9: note = Description of Artificial Sequence: Synthetic peptide
AETSHVPWT

SEQ ID NO: 123 - protein, 9 aa, synthetic construct
  REGION 1..9: note = Description of Artificial Sequence: Synthetic peptide
SQSSIYPWT

SEQ ID NO: 124 - protein, 117 aa, synthetic construct
  REGION 1..117: note = Description of Artificial Sequence: Synthetic polypeptide
QIQLVQSGPELKKPGETVKISCKASGYTFTDYSINWVKRAPGKGLKWMGWINTETREPAYAYDFRGRFAFSLETSASTAYLQINNLKYEDTATYFCALDYSYAMDYWGQGTSVTVSS

SEQ ID NO: 125 - protein, 5 aa, synthetic construct
  REGION 1..5: note = Description of Artificial Sequence: Synthetic peptide
DYSIN

SEQ ID NO: 126 - protein, 16 aa, synthetic construct
  REGION 1..16: note = Description of Artificial Sequence: Synthetic peptide
WINTETREPAYAYDFR

SEQ ID NO: 127 - protein, 8 aa, synthetic construct
  REGION 1..8: note = Description of Artificial Sequence: Synthetic peptide
DYSYAMDY

SEQ ID NO: 128 - protein, 111 aa, synthetic construct
  REGION 1..111: note = Description of Artificial Sequence: Synthetic polypeptide
DIVLTQSPPSLAMSLGKRATISCRASESVTILGSHLIHWYQQKPGQPPTLLIQLASNVQTGVPARFSGSGSRTDFTLTIDPVEEDDVAVYYCLQSRTIPRTFGGGTKLEIK

SEQ ID NO: 129 - protein, 15 aa, synthetic construct
  REGION 1..15: note = Description of Artificial Sequence: Synthetic peptide
RASESVTILGSHLIH

SEQ ID NO: 130 - protein, 7 aa, synthetic construct
  REGION 1..7: note = Description of Artificial Sequence: Synthetic peptide
LASNVQT

SEQ ID NO: 131 - protein, 9 aa, synthetic construct
  REGION 1..9: note = Description of Artificial Sequence: Synthetic peptide
LQSRTIPRT

SEQ ID NO: 132 - protein, 121 aa, synthetic construct
  REGION 1..121: note = Description of Artificial Sequence: Synthetic polypeptide
QVQLVQSGAEVKKPGSSVKVSCKASGGTFSNYWMHWVRQAPGQGLEWMGATYRGHSDTYYNQKFKGRVTITADKSTSTAYMELSSLRSEDTAVYYCARGAIYNGYDVLDNWGQGTLVTVSS

SEQ ID NO: 133 - protein, 5 aa, synthetic construct
  REGION 1..5: note = Description of Artificial Sequence: Synthetic peptide
NYWMH

SEQ ID NO: 134 - protein, 17 aa, synthetic construct
  REGION 1..17: note = Description of Artificial Sequence: Synthetic peptide
ATYRGHSDTYYNQKFKG

SEQ ID NO: 135 - protein, 12 aa, synthetic construct
  REGION 1..12: note = Description of Artificial Sequence: Synthetic peptide
GAIYNGYDVLDN

SEQ ID NO: 136 - protein, 108 aa, synthetic construct
  REGION 1..108: note = Description of Artificial Sequence: Synthetic polypeptide
DIQMTQSPSSLSASVGDRVTITCSASQDISNYLNWYQQKPGKAPKLLIYYTSNLHSGVPSRFSGSGSGTDFTLTISSLQPEDFATYYCQQYRKLPWTFGQGTKLEIKR

SEQ ID NO: 137 - protein, 11 aa, synthetic construct
  REGION 1..11: note = Description of Artificial Sequence: Synthetic peptide
SASQDISNYLN

SEQ ID NO: 138 - protein, 7 aa, synthetic construct
  REGION 1..7: note = Description of Artificial Sequence: Synthetic peptide
YTSNLHS

SEQ ID NO: 139 - protein, 9 aa, synthetic construct
  REGION 1..9: note = Description of Artificial Sequence: Synthetic peptide
QQYRKLPWT

SEQ ID NO: 140 - protein, 121 aa, synthetic construct
  REGION 1..121: note = Description of Artificial Sequence: Synthetic polypeptide
QLQLQESGPGLVKPSETLSLTCTVSGGSISSSSYFWGWIRQPPGKGLEWIGSIYYSGITYYNPSLKSRVTISVDTSKNQFSLKLSSVTAADTAVYYCARHDGATAGLFDYWGQGTLVTVSS

SEQ ID NO: 141 - protein, 7 aa, synthetic construct
  REGION 1..7: note = Description of Artificial Sequence: Synthetic peptide
SSSYFWG

SEQ ID NO: 142 - protein, 16 aa, synthetic construct
  REGION 1..16: note = Description of Artificial Sequence: Synthetic peptide
SIYYSGITYYNPSLKS

SEQ ID NO: 143 - protein, 11 aa, synthetic construct
  REGION 1..11: note = Description of Artificial Sequence: Synthetic peptide
HDGATAGLFDY

SEQ ID NO: 144 - protein, 108 aa, synthetic construct
  REGION 1..108: note = Description of Artificial Sequence: Synthetic polypeptide
SYVLTQPPSVSVAPGQTARITCGGNNIGSKSVHWYQQPPGQAPVVVVYDDSDRPSGIPERFSGSNSGNTATLTISRVEAGDEAVYYCQVWDSSSDHVVFGGGTKLTVL

SEQ ID NO: 145 - protein, 11 aa, synthetic construct
  REGION 1..11: note = Description of Artificial Sequence: Synthetic peptide
GGNNIGSKSVH

SEQ ID NO: 146 - protein, 7 aa, synthetic construct
  REGION 1..7: note = Description of Artificial Sequence: Synthetic peptide
DDSDRPS

SEQ ID NO: 147 - protein, 11 aa, synthetic construct
  REGION 1..11: note = Description of Artificial Sequence: Synthetic peptide
QVWDSSSDHVV

SEQ ID NO: 148 - protein, 116 aa, synthetic construct
  REGION 1..116: note = Description of Artificial Sequence: Synthetic polypeptide
EVQLLESGGGLVQPGGSLRLSCAASGFTFSDNAMGWVRQAPGKGLEWVSAISGPGSSTYYADSVKGRFTISRDNSKNTLYLQMNSLRAEDTAVYYCAKVLGWFDYWGQGTLVTVSS

SEQ ID NO: 149 - protein, 12 aa, synthetic construct
  REGION 1..12: note = Description of Artificial Sequence: Synthetic peptide
RASQSVSDEYLS

SEQ ID NO: 150 - protein, 7 aa, synthetic construct
  REGION 1..7: note = Description of Artificial Sequence: Synthetic peptide
SASTRAT

SEQ ID NO: 151 - protein, 10 aa, synthetic construct
  REGION 1..10: note = Description of Artificial Sequence: Synthetic peptide
QQYGYPPDFT

SEQ ID NO: 152 - protein, 109 aa, synthetic construct
  REGION 1..109: note = Description of Artificial Sequence: Synthetic polypeptide
EIVLTQSPGTLSLSPGERATLSCRASQSVSDEYLSWYQQKPGQAPRLLIHSASTRATGIPDRFSGSGSGTDFTLAISRLEPEDFAVYYCQQYGYPPDFTFGQGTKVEIK

SEQ ID NO: 153 - protein, 12 aa, synthetic construct
  REGION 1..12: note = Description of Artificial Sequence: Synthetic peptide
RASQSVSDEYLS

SEQ ID NO: 154 - protein, 7 aa, synthetic construct
  REGION 1..7: note = Description of Artificial Sequence: Synthetic peptide
SASTRAT

SEQ ID NO: 155 - protein, 10 aa, synthetic construct
  REGION 1..10: note = Description of Artificial Sequence: Synthetic peptide
QQYGYPPDFT

SEQ ID NO: 156 - protein, 184 aa, Homo sapiens
MLQMAGQCSQNEYFDSLLHACIPCQLRCSSNTPPLTCQRYCNASVTNSVKGTNAILWTCLGLSLIISLAVFVLMFLLRKINSEPLKDEFKNTGSGLLGMANIDLEKSRTGDEIILPRGLEYTVEECTCEDCIKSKPKVDSDHCFPLPAMEEGATILVTTKTNDYCKSLPAALSATEIEKSISAR

SEQ ID NO: 157 - protein, 116 aa, synthetic construct
  REGION 1..116: note = Description of Artificial Sequence: Synthetic polypeptide
EVQLLESGGGLVQPGGSLRLSCAASGFTFSSYAMSWVRQAPGKGLEWVSAISGSGGSTYYADSVKGRFTISRDNSKNTLYLQMNSLRAEDTAVYYCAKVLGWFDYWGQGTLVTVSS

SEQ ID NO: 158 - protein, 109 aa, synthetic construct
  REGION 1..109: note = Description of Artificial Sequence: Synthetic polypeptide
EIVLTQSPGTLSLSPGERATLSCRASQSVSSSYLAWYQQKPGQAPRLLIYGASSRATGIPDRFSGSGSGTDFTLTISRLEPEDFAVYYCQQYGYPPDFTFGQGTKVEIK

SEQ ID NO: 159 - protein, 116 aa, synthetic construct; identical to SEQ ID NO: 148
  REGION 1..116: note = Description of Artificial Sequence: Synthetic polypeptide

SEQ ID NO: 160 - protein, 109 aa, synthetic construct; identical to SEQ ID NO: 152
  REGION 1..109: note = Description of Artificial Sequence: Synthetic polypeptide

SEQ ID NO: 161 - protein, 128 aa, synthetic construct
  REGION 1..128: note = Description of Artificial Sequence: Synthetic polypeptide
EVQLVESGGGLVQPGGSLRLSCAASGFTFSSYGMSWVRQAPGKGLEWVANIKQDGSEKYYVDSVKGRFTISRDNAKNSLYLQMNSLRAEDTAVYYCAREGGPYYDSSGYFVYYGMDVWGQGTTVTVSS

SEQ ID NO: 162 - protein, 9 aa, synthetic construct
  REGION 1..9: note = Description of Artificial Sequence: Synthetic peptide
FTFSSYGMS

SEQ ID NO: 163 - protein, 17 aa, synthetic construct
  REGION 1..17: note = Description of Artificial Sequence: Synthetic peptide
NIKQDGSEKYYVDSVKG

SEQ ID NO: 164 - protein, 21 aa, synthetic construct
  REGION 1..21: note = Description of Artificial Sequence: Synthetic peptide
AREGGPYYDSSGYFVYYGMDV

SEQ ID NO: 165 - protein, 106 aa, synthetic construct
  REGION 1..106: note = Description of Artificial Sequence: Synthetic polypeptide
DIQMTQSPSTLSASVGDRVTITCRASQSISSWLAWYQQKPGKAPKLLIYDASSLESGVPSRFSGSGSGTEFTLTISSLQPDDFATYYCQQYESFPTFGGGTKVEIK

SEQ ID NO: 166 - protein, 11 aa, synthetic construct
  REGION 1..11: note = Description of Artificial Sequence: Synthetic peptide
RASQSISSWLA

SEQ ID NO: 167 - protein, 7 aa, synthetic construct
  REGION 1..7: note = Description of Artificial Sequence: Synthetic peptide
DASSLES

SEQ ID NO: 168 - protein, 8 aa, synthetic construct
  REGION 1..8: note = Description of Artificial Sequence: Synthetic peptide
QQYESFPT

SEQ ID NO: 169 - protein, 118 aa, synthetic construct
  REGION 1..118: note = Description of Artificial Sequence: Synthetic polypeptide
EVQLVESGGGLVQPGGSLRLSCAASGFTFSSYWMSWVRQAPGKGLEWVANIKQDGSEKYYVDSVKGRFTISRDNAKNSLYLQMNSLRAEDTAVYYCARPLNAGELDVWGQGTMVTVSS

SEQ ID NO: 170 - protein, 9 aa, synthetic construct
  REGION 1..9: note = Description of Artificial Sequence: Synthetic peptide
FTFSSYWMS

SEQ ID NO: 171 - protein, 17 aa, synthetic construct
  REGION 1..17: note = Description of Artificial Sequence: Synthetic peptide
NIKQDGSEKYYVDSVKG

SEQ ID NO: 172 - protein, 11 aa, synthetic construct
  REGION 1..11: note = Description of Artificial Sequence: Synthetic peptide
ARPLNAGELDV

SEQ ID NO: 173 - protein, 107 aa, synthetic construct
  REGION 1..107: note = Description of Artificial Sequence: Synthetic polypeptide
DIQMTQSPSTLSASVGDRVTITCRASQSISSWLAWYQQKPGKAPKLLIYEASSLESGVPSRFSGSGSGTEFTLTISSLQPDDFATYYCQQLESYPLTFGGGTKVEIK

SEQ ID NO: 174 - protein, 11 aa, synthetic construct
  REGION 1..11: note = Description of Artificial Sequence: Synthetic peptide
RASQSISSWLA

SEQ ID NO: 175 - protein, 7 aa, synthetic construct
  REGION 1..7: note = Description of Artificial Sequence: Synthetic peptide
EASSLES

SEQ ID NO: 176 - protein, 9 aa, synthetic construct
  REGION 1..9: note = Description of Artificial Sequence: Synthetic peptide
QQLESYPLT

SEQ ID NO: 177 - protein, 128 aa, synthetic construct
  REGION 1..128: note = Description of Artificial Sequence: Synthetic polypeptide
EVQLLESGGGLVQPGGSLRLSCAASGFTFSKYTMSWVRQAPGKGLEWVSAIVGSGESTYFADSVKGRFTISRDNSKNTLYLQMNSLRAEDTAVYYCAREGGPYYDSSGYFVYYGMDVWGQGTTVTVSS

SEQ ID NO: 178 - protein, 9 aa, synthetic construct
  REGION 1..9: note = Description of Artificial Sequence: Synthetic peptide
FTFSKYTMS

SEQ ID NO: 179 - protein, 17 aa, synthetic construct
  REGION 1..17: note = Description of Artificial Sequence: Synthetic peptide
AIVGSGESTYFADSVKG

SEQ ID NO: 180 - protein, 21 aa, synthetic construct
  REGION 1..21: note = Description of Artificial Sequence: Synthetic peptide
AREGGPYYDSSGYFVYYGMDV

SEQ ID NO: 181 - protein, 106 aa, synthetic construct
  REGION 1..106: note = Description of Artificial Sequence: Synthetic polypeptide
DIQMTQSPSTLSASVGDRVTITCRASQSISSWLAWYQQKPGKAPKLLIYKASSLESGVPSRFSGSGSGTEFTLTISSLQPDDFATYYCQQYDDLPTFGGGTKVEIK

SEQ ID NO: 182 - protein, 11 aa, synthetic construct
  REGION 1..11: note = Description of Artificial Sequence: Synthetic peptide
RASQSISSWLA

SEQ ID NO: 183 - protein, 7 aa, synthetic construct
  REGION 1..7: note = Description of Artificial Sequence: Synthetic peptide
KASSLES

SEQ ID NO: 184 - protein, 8 aa, synthetic construct
  REGION 1..8: note = Description of Artificial Sequence: Synthetic peptide
QQYDDLPT

SEQ ID NO: 185 - protein, 123 aa, synthetic construct
  REGION 1..123: note = Description of Artificial Sequence: Synthetic polypeptide
QVQLVQSGAEVKKPGASVKVSCKASGYTFSDYYMHWVRQAPGQGLEWMGMINPSWGSTSYAQKFQGRVTMTRDTSTSTVYMELSSLRSEDTAVYYCAREAADGFVGERYFDLWGRGTLVTVSS

SEQ ID NO: 186 - protein, 9 aa, synthetic construct
  REGION 1..9: note = Description of Artificial Sequence: Synthetic peptide
YTFSDYYMH

SEQ ID NO: 187 - protein, 17 aa, synthetic construct
  REGION 1..17: note = Description of Artificial Sequence: Synthetic peptide
MINPSWGSTSYAQKFQG

SEQ ID NO: 188 - protein, 16 aa, synthetic construct
  REGION 1..16: note = Description of Artificial Sequence: Synthetic peptide
AREAADGFVGERYFDL

SEQ ID NO: 189 - protein, 112 aa, synthetic construct
  REGION 1..112: note = Description of Artificial Sequence: Synthetic polypeptide
DIVMTQSPLSLPVTPGEPASISCRSSQSLLYSNGYNYLDWYLQKPGQSPQLLIYLGSNRASGVPDRFSGSGSGTDFTLKISRVEAEDVGVYYCMQDVALPITFGGGTKVEIK

SEQ ID NO: 190 - protein, 16 aa, synthetic construct
  REGION 1..16: note = Description of Artificial Sequence: Synthetic peptide
RSSQSLLYSNGYNYLD

SEQ ID NO: 191 - protein, 7 aa, synthetic construct
  REGION 1..7: note = Description of Artificial Sequence: Synthetic peptide
LGSNRAS

SEQ ID NO: 192 - protein, 9 aa, synthetic construct
  REGION 1..9: note = Description of Artificial Sequence: Synthetic peptide
MQDVALPIT

SEQ ID NO: 193 - protein, 118 aa, synthetic construct
  REGION 1..118: note = Description of Artificial Sequence: Synthetic polypeptide
EVQLVESGGGLVQPGGSLRLSCAASGFTFGSYWMSWVRQAPGKGLEWVATIKQDGSEKSYVDSVKGRFTISRDNAKNSLYLQMNSLRAEDTAVYYCARPLNAGELDVWGQGTMVTVSS

SEQ ID NO: 194 - protein, 9 aa, synthetic construct
  REGION 1..9: note = Description of Artificial Sequence: Synthetic peptide
FTFGSYWMS

SEQ ID NO: 195 - protein, 17 aa, synthetic construct
  REGION 1..17: note = Description of Artificial Sequence: Synthetic peptide
TIKQDGSEKSYVDSVKG

SEQ ID NO: 196 - protein, 11 aa, synthetic construct
  REGION 1..11: note = Description of Artificial Sequence: Synthetic peptide
ARPLNAGELDV

SEQ ID NO: 197 - protein, 108 aa, synthetic construct
  REGION 1..108: note = Description of Artificial Sequence: Synthetic polypeptide
DIQMTQSPSTLSASVGDRVTITCRASQSISSWLAWYQQKPGKAPKLLIYEASSLESGVPSRFSGSGSGTEFTLTISSLQPDDFATYYCQQSQSYPPITFGGGTKVEIK

SEQ ID NO: 198 - protein, 11 aa, synthetic construct
  REGION 1..11: note = Description of Artificial Sequence: Synthetic peptide
RASQSISSWLA

SEQ ID NO: 199 - protein, 7 aa, synthetic construct
  REGION 1..7: note = Description of Artificial Sequence: Synthetic peptide
EASSLES

SEQ ID NO: 200 - protein, 10 aa, synthetic construct
  REGION 1..10: note = Description of Artificial Sequence: Synthetic peptide
QQSQSYPPIT

SEQ ID NO: 201 - protein, 118 aa, synthetic construct
  REGION 1..118: note = Description of Artificial Sequence: Synthetic polypeptide
EVQLVESGGGLVQPGGSLRLSCAASGFTFPSYWMSWVRQAPGKGLEWVATIKRDGSEKGYVDSVKGRFTISRDNAKNSLYLQMNSLRAEDTAVYYCARPLNAGELDVWGQGTMVTVSS

SEQ ID NO: 202 - protein, 9 aa, synthetic construct
  REGION 1..9: note = Description of Artificial Sequence: Synthetic peptide
FTFPSYWMS

SEQ ID NO: 203 - protein, 17 aa, synthetic construct
  REGION 1..17: note = Description of Artificial Sequence: Synthetic peptide
TIKRDGSEKGYVDSVKG

SEQ ID NO: 204 - protein, 11 aa, synthetic construct
  REGION 1..11: note = Description of Artificial Sequence: Synthetic peptide
ARPLNAGELDV

SEQ ID NO: 205 - protein, 108 aa, synthetic construct; identical to SEQ ID NO: 197
  REGION 1..108: note = Description of Artificial Sequence: Synthetic polypeptide

SEQ ID NO: 206 - protein, 11 aa, synthetic construct
  REGION 1..11: note = Description of Artificial Sequence: Synthetic peptide
RASQSISSWLA

SEQ ID NO: 207 - protein, 7 aa, synthetic construct
  REGION 1..7: note = Description of Artificial Sequence: Synthetic peptide
EASSLES

SEQ ID NO: 208 - protein, 10 aa, synthetic construct
  REGION 1..10: note = Description of Artificial Sequence: Synthetic peptide
QQSQSYPPIT

SEQ ID NO: 209 - protein, 120 aa, synthetic construct
  REGION 1..120: note = Description of Artificial Sequence: Synthetic polypeptide
QVQLVQSGAEVKKPGASVKVSCKASGYTFGTYYMHWVRQAPGQGLEWMGIINPSRGSTVYAQKFQGRVTMTRDTSTSTVYMELSSLRSEDTAVYYCARGAGYDDEDMDVWGKGTTVTVSS

SEQ ID NO: 210 - protein, 9 aa, synthetic construct
  REGION 1..9: note = Description of Artificial Sequence: Synthetic peptide
YTFGTYYMH

SEQ ID NO: 211 - protein, 17 aa, synthetic construct
  REGION 1..17: note = Description of Artificial Sequence: Synthetic peptide
IINPSRGSTVYAQKFQG

SEQ ID NO: 212 - protein, 13 aa, synthetic construct
  REGION 1..13: note = Description of Artificial Sequence: Synthetic peptide
ARGAGYDDEDMDV

SEQ ID NO: 213 - protein, 107 aa, synthetic construct
  REGION 1..107: note = Description of Artificial Sequence: Synthetic polypeptide
DIQMTQSPSSVSASVGDRVTITCRASQGIDSWLAWYQQKPGKAPKLLIYAASSLQSGVPSRFSGSGSGTDFTLTISSLQPEDFATYYCQQAHSYPLTFGGGTKVEIK

SEQ ID NO: 214 - protein, 11 aa, synthetic construct
  REGION 1..11: note = Description of Artificial Sequence: Synthetic peptide
RASQGIDSWLA

SEQ ID NO: 215 - protein, 7 aa, synthetic construct
  REGION 1..7: note = Description of Artificial Sequence: Synthetic peptide
AASSLQS

SEQ ID NO: 216 - protein, 9 aa, synthetic construct
  REGION 1..9: note = Description of Artificial Sequence: Synthetic peptide
QQAHSYPLT

SEQ ID NO: 217 - protein, 128 aa, synthetic construct
  REGION 1..128: note = Description of Artificial Sequence: Synthetic polypeptide
EVQLVESGGGLVKPGGSLRLSCAASGFTFSSYAMSWVRQAPGKGLEWVSSISSSSEGIYYADSVKGRFTISRDNAKNSLYLQMNSLRAEDTAVYYCAREGGPYYDSSGYFVYYGMDVWGQGTTVTVSS

SEQ ID NO: 218 - protein, 9 aa, synthetic construct
  REGION 1..9: note = Description of Artificial Sequence: Synthetic peptide
FTFSSYAMS

SEQ ID NO: 219 - protein, 17 aa, synthetic construct
  REGION 1..17: note = Description of Artificial Sequence: Synthetic peptide
SISSSSEGIYYADSVKG

SEQ ID NO: 220 - protein, 21 aa, synthetic construct
  REGION 1..21: note = Description of Artificial Sequence: Synthetic peptide
AREGGPYYDSSGYFVYYGMDV

SEQ ID NO: 221 - protein, 106 aa, synthetic construct
  REGION 1..106: note = Description of Artificial Sequence: Synthetic polypeptide
DIQMTQSPSTLSASVGDRVTITCRASNSISSWLAWYQQKPGKAPKLLIYEASSTKSGVPSRFSGSGSGTEFTLTISSLQPDDFATYYCQQYDDLPTFGGGTKVEIK

SEQ ID NO: 222 - protein, 11 aa, synthetic construct
  REGION 1..11: note = Description of Artificial Sequence: Synthetic peptide
RASNSISSWLA

SEQ ID NO: 223 - protein, 7 aa, synthetic construct
  REGION 1..7: note = Description of Artificial Sequence: Synthetic peptide
EASSTKS

SEQ ID NO: 224 - protein, 8 aa, synthetic construct
  REGION 1..8: note = Description of Artificial Sequence: Synthetic peptide
QQYDDLPT

SEQ ID NO: 225 - protein, 123 aa, synthetic construct
  REGION 1..123: note = Description of Artificial Sequence: Synthetic polypeptide
EVQLVESGGGLVQPGGSLRLSCAASGFTFSSYWMSWVRQAPGKGLEWVANINTDGSEVYYVDSVKGRFTISRDNAKNSLYLQMNSLRAEDTAVYYCARDVGPGIAYQGHFDYWGQGTLVTVSS

SEQ ID NO: 226 - protein, 9 aa, synthetic construct
  REGION 1..9: note = Description of Artificial Sequence: Synthetic peptide
FTFSSYWMS

SEQ ID NO: 227 - protein, 17 aa, synthetic construct
  REGION 1..17: note = Description of Artificial Sequence: Synthetic peptide
NINTDGSEVYYVDSVKG

SEQ ID NO: 228 - protein, 16 aa, synthetic construct
  REGION 1..16: note = Description of Artificial Sequence: Synthetic peptide
ARDVGPGIAYQGHFDY

SEQ ID NO: 229 - protein, 107 aa, synthetic construct
  REGION 1..107: note = Description of Artificial Sequence: Synthetic polypeptide
DIQMTQSPSSLSASVGDRVTITCRASQVIYSYLNWYQQKPGKAPKLLIYAASSLKSGVPSRFSGSGSGTDFTLTISSLQPEDFATYYCQQVYDTPLTFGGGTKVEIK

SEQ ID NO: 230 - protein, 11 aa, synthetic construct
  REGION 1..11: note = Description of Artificial Sequence: Synthetic peptide
RASQVIYSYLN

SEQ ID NO: 231 - protein, 7 aa, synthetic construct
  REGION 1..7: note = Description of Artificial Sequence: Synthetic peptide
AASSLKS

SEQ ID NO: 232 - protein, 9 aa, synthetic construct
  REGION 1..9: note = Description of Artificial Sequence: Synthetic peptide
QQVYDTPLT

SEQ ID NO: 233 - protein, 120 aa, synthetic construct
  REGION 1..120: note = Description of Artificial Sequence: Synthetic polypeptide
QLQLQESGPGLVKPSETLSLTCTVSGGSISSTDYYWGWIRQPPGKGLEWIGSIGYSGTYYNPSLKSRVTISVDTSKNQFSLKLSSVTAADTAVYYCARETAHDVHGMDVWGQGTTVTVSS

SEQ ID NO: 234 - protein, 11 aa, synthetic construct
  REGION 1..11: note = Description of Artificial Sequence: Synthetic peptide
GSISSTDYYWG

SEQ ID NO: 235 - protein, 15 aa, synthetic construct
  REGION 1..15: note = Description of Artificial Sequence: Synthetic peptide
SIGYSGTYYNPSLKS

SEQ ID NO: 236 - protein, 13 aa, synthetic construct
  REGION 1..13: note = Description of Artificial Sequence: Synthetic peptide
ARETAHDVHGMDV

SEQ ID NO: 237 - protein, 106 aa, synthetic construct
  REGION 1..106: note = Description of Artificial Sequence: Synthetic polypeptide
EIVLTQSPATLSLSPGERATLSCRASHSVYSYLAWYQQKPGQAPRLLIYDASNRATGIPARFSGSGSGTDFTLTISSLEPEDFAVYYCQQYDNLPTFGGGTKVEIK

SEQ ID NO: 238 - protein, 11 aa, synthetic construct
  REGION 1..11: note = Description of Artificial Sequence: Synthetic peptide
RASHSVYSYLA

SEQ ID NO: 239 - protein, 7 aa, synthetic construct
  REGION 1..7: note = Description of Artificial Sequence: Synthetic peptide
DASNRAT

SEQ ID NO: 240 - protein, 8 aa, synthetic construct
  REGION 1..8: note = Description of Artificial Sequence: Synthetic peptide
QQYDNLPT

SEQ ID NO: 241 - protein, 116 aa, synthetic construct
  REGION 1..116: note = Description of Artificial Sequence: Synthetic polypeptide
QVQLVQSGAEVKKPGSSVKVSCKASGYTFTDYNMHWVRQAPGQGLEWIGYIYPYNGGTGYNQKFKSKATITADESTNTAYMELSSLRSEDTAVYYCARGRPAMDYWGQGTLVTVSS

SEQ ID NO: 242 - protein, 7 aa, synthetic construct
  REGION 1..7: note = Description of Artificial Sequence: Synthetic peptide
GYTFTDY

SEQ ID NO: 243 - protein, 10 aa, synthetic construct
  REGION 1..10: note = Description of Artificial Sequence: Synthetic peptide
YIYPYNGGTG

SEQ ID NO: 244 - protein, 7 aa, synthetic construct
  REGION 1..7: note = Description of Artificial Sequence: Synthetic peptide
GRPAMDY

SEQ ID NO: 245 - protein, 111 aa, synthetic construct
  REGION 1..111: note = Description of Artificial Sequence: Synthetic polypeptide
DIQMTQSPSSLSASVGDRVTITCRASESVDNYGISFMNWFQQKPGKAPKLLIYAASNQGSGVPSRFSGSGSGTDFTLTISSLQPDDFATYYCQQSKEVPWTFGQGTKVEIK

SEQ ID NO: 246 - protein, 12 aa, synthetic construct
  REGION 1..12: note = Description of Artificial Sequence: Synthetic peptide
ESVDNYGISFMN

SEQ ID NO: 247 - protein, 7 aa, synthetic construct
  REGION 1..7: note = Description of Artificial Sequence: Synthetic peptide
AASNQGS

SEQ ID NO: 248 - protein, 9 aa, synthetic construct
  REGION 1..9: note = Description of Artificial Sequence: Synthetic peptide
QQSKEVPWT

SEQ ID NO: 249 - protein, 116 aa, synthetic construct [sequence omitted]

SEQ ID NO: 250 - protein, 7 aa, synthetic construct
  REGION 1..7: note = Description of Artificial Sequence: Synthetic peptide
GYTITDS

SEQ ID NO: 251 - protein, 10 aa, synthetic construct
  REGION 1..10: note = Description of Artificial Sequence: Synthetic peptide
YIYPYNGGTD

SEQ ID NO: 252 - protein, 7 aa, synthetic construct
  REGION 1..7: note = Description of Artificial Sequence: Synthetic peptide
GNPWLAY

SEQ ID NO: 253 - protein, 111 aa, synthetic construct [sequence omitted]

SEQ ID NO: 254 - protein, 12 aa, synthetic construct
  REGION 1..12: note = Description of Artificial Sequence: Synthetic peptide
ESLDNYGIRFLT

SEQ ID NO: 255 - protein, 7 aa, synthetic construct
  REGION 1..7: note = Description of Artificial Sequence: Synthetic peptide
AASNQGS

SEQ ID NO: 256 - protein, 9 aa, synthetic construct
  REGION 1..9: note = Description of Artificial Sequence: Synthetic peptide
QQTKEVPWS

SEQ ID NO: 257 - protein, 118 aa, synthetic construct
  REGION 1..118: note = Description of Artificial Sequence: Synthetic polypeptide
QVQLQQPGAEVVKPGASVKMSCKASGYTFTSYYIHWIKQTPGQGLEWVGVIYPGNDDISYNQKFQGKATLTADKSSTTAYMQLSSLTSEDSAVYYCAREVRLRYFDVWGQGTTVTVSS

SEQ ID NO: 258 - protein, 7 aa, synthetic construct
  REGION 1..7: note = Description of Artificial Sequence: Synthetic peptide
GYTFTSY

SEQ ID NO: 259 - protein, 6 aa, synthetic construct
  REGION 1..6: note = Description of Artificial Sequence: Synthetic peptide
YPGNDD

SEQ ID NO: 260 - protein, 9 aa, synthetic construct
  REGION 1..9: note = Description of Artificial Sequence: Synthetic peptide
EVRLRYFDV

SEQ ID NO: 261 - protein, 113 aa, synthetic construct
  REGION 1..113: note = Description of Artificial Sequence: Synthetic polypeptide
EIVLTQSPGSLAVSPGERVTMSCKSSQSVFFSSSQKNYLAWYQQIPGQSPRLLIYWASTRESGVPDRFTGSGSGTDFTLTISSVQPEDLAIYYCHQYLSSRTFGQGTKLEIKR

SEQ ID NO: 262 - protein, 14 aa, synthetic construct
  REGION 1..14: note = Description of Artificial Sequence: Synthetic peptide
QSVFFSSSQKNYLA

SEQ ID NO: 263 - protein, 7 aa, synthetic construct
  REGION 1..7: note = Description of Artificial Sequence: Synthetic peptide
WASTRES

SEQ ID NO: 264 - protein, 8 aa, synthetic construct
  REGION 1..8: note = Description of Artificial Sequence: Synthetic peptide
HQYLSSRT

SEQ ID NO: 265 - protein, 118 aa, synthetic construct
  REGION 1..118: note = Description of Artificial Sequence: Synthetic polypeptide
QVQLVQSGAEVKKPGASVKVSCKASGYTFTNYDINWVRQAPGQGLEWIGWIYPGDGSTKYNEKFKAKATLTADTSTSTAYMELRSLRSDDTAVYYCASGYEDAMDYWGQGTTVTVSSA

SEQ ID NO: 266 - protein, 7 aa, synthetic construct
  REGION 1..7: note = Description of Artificial Sequence: Synthetic peptide
GYTFTNY

SEQ ID NO: 267 - protein, 6 aa, synthetic construct
  REGION 1..6: note = Description of Artificial Sequence: Synthetic peptide
YPGDGS

SEQ ID NO: 268 - protein, 8 aa, synthetic construct
  REGION 1..8: note = Description of Artificial Sequence: Synthetic peptide
GYEDAMDY

SEQ ID NO: 269 - protein, 108 aa, synthetic construct
  REGION 1..108: note = Description of Artificial Sequence: Synthetic polypeptide
DIQMTQSPSSLSASVGDRVTINCKASQDINSYLSWFQQKPGKAPKTLIYRANRLVDGVPSRFSGSGSGQDYTLTISSLQPEDFATYYCLQYDEFPLTFGGGTKVEIKR

SEQ ID NO: 270 - protein, 8 aa, synthetic construct
  REGION 1..8: note = Description of Artificial Sequence: Synthetic peptide
QDINSYLS

SEQ ID NO: 271 - protein, 7 aa, synthetic construct
  REGION 1..7: note = Description of Artificial Sequence: Synthetic peptide
RANRLVD

SEQ ID NO: 272 - protein, 9 aa, synthetic construct
  REGION 1..9: note = Description of Artificial Sequence: Synthetic peptide
LQYDEFPLT

SEQ ID NO: 273 - protein, 364 aa, Homo sapiens
MPLLLLLPLLWAGALAMDPNFWLQVQESVTVQEGLCVLVPCTFFHPIPYYDKNSPVHGYWFREGAIISRDSPVATNKLDQEVQEETQGRFRLLGDPSRNNCSLSIVDARRRDNGSYFFRMERGSTKYSYKSPQLSVHVTDLTHRPKILIPGTLEPGHSKNLTCSVSWACEQGTPPIFSWLSAAPTSLGPRTTHSSVLIITPRPQDHGTNLTCQVKFAGAGVTTERTIQLNVTYVPQNPTTGIFPGDGSGKQETRAGVVHGAIGGAGVTALLALCLCLIFFIVKTHRRKAARTAVGRNDTHPTTGSASPKHQKKSKLHGPTETSSCSGAAPTVEMDEELHYASLNFHGMNPSKDTSTEYSEVRTQ

SEQ ID NO: 274 - protein, 120 aa, synthetic construct [sequence omitted]

SEQ ID NO: 275 - protein, 7 aa, synthetic construct
  REGION 1..7: note = Description of Artificial Sequence: Synthetic peptide
GFNIKDT

SEQ ID NO: 276 - protein, 6 aa, synthetic construct
  REGION 1..6: note = Description of Artificial Sequence: Synthetic peptide
YPTNGY

SEQ ID NO: 277 - protein, 11 aa, synthetic construct
  REGION 1..11: note = Description of Artificial Sequence: Synthetic peptide
WGGDGFYAMDY

SEQ ID NO: 278 - protein, 107 aa, synthetic construct [sequence omitted]

SEQ ID NO: 279 - protein, 8 aa, synthetic construct
  REGION 1..8: note = Description of Artificial Sequence: Synthetic peptide
QDVNTAVA

SEQ ID NO: 280 - protein, 7 aa, synthetic construct
  REGION 1..7: note = Description of Artificial Sequence: Synthetic peptide
SASFLYS

SEQ ID NO: 281 - protein, 9 aa, synthetic construct
  REGION 1..9: note = Description of Artificial Sequence: Synthetic peptide
QQHYTTPPT

SEQ ID NO: 282 - protein, 120 aa, synthetic construct
  REGION 1..120: note = Description of Artificial Sequence: Synthetic polypeptide
EVQLVESGGGLVQPGGSLRLSCAASGFTFTDYTMDWVRQAPGKGLEWVADVNPNSGGSIYNQRFKGRFTLSVDRSKNTLYLQMNSLRAEDTAVYYCARNLGPSFYFDYWGQGTLVTVSSA

SEQ ID NO: 283 - protein, 7 aa, synthetic construct
  REGION 1..7: note = Description of Artificial Sequence: Synthetic peptide
GFTFTDY

SEQ ID NO: 284 - protein, 6 aa, synthetic construct
  REGION 1..6: note = Description of Artificial Sequence: Synthetic peptide
NPNSGG

SEQ ID NO: 285 - protein, 10 aa, synthetic construct
  REGION 1..10: note = Description of Artificial Sequence: Synthetic peptide
NLGPSFYFDY

SEQ ID NO: 286 - protein, 108 aa, synthetic construct
  REGION 1..108: note = Description of Artificial Sequence: Synthetic polypeptide
DIQMTQSPSSLSASVGDRVTITCKASQDVSIGVAWYQQKPGKAPKLLIYSASYRYTGVPSRFSGSGSGTDFTLTISSLQPEDFATYYCQQYYIYPYTFGQGTKVEIKR

SEQ ID NO: 287 - protein, 8 aa, synthetic construct
  REGION 1..8: note = Description of Artificial Sequence: Synthetic peptide
QDVSIGVA

SEQ ID NO: 288 - protein, 7 aa, synthetic construct
  REGION 1..7: note = Description of Artificial Sequence: Synthetic peptide
SASYRYT

SEQ ID NO: 289 - protein, 9 aa, synthetic construct
  REGION 1..9: note = Description of Artificial Sequence: Synthetic peptide
QQYYIYPYT

SEQ ID NO: 290 - protein, 121 aa, synthetic construct
  REGION 1..121: note = Description of Artificial Sequence: Synthetic polypeptide
QVQLQQSGPELVKPGASLKLSCTASGFNIKDTYIHWVKQRPEQGLEWIGRIYPTNGYTRYDPKFQDKATITADTSSNTAYLQVSRLTSEDTAVYYCSRWGGDGFYAMDYWGQGASVTVSSA

SEQ ID NO: 291 - protein, 7 aa, synthetic construct
  REGION 1..7: note = Description of Artificial Sequence: Synthetic peptide
GFNIKDT

SEQ ID NO: 292 - protein, 6 aa, synthetic construct
  REGION 1..6: note = Description of Artificial Sequence: Synthetic peptide
YPTNGY

SEQ ID NO: 293 - protein, 11 aa, synthetic construct
  REGION 1..11: note = Description of Artificial Sequence: Synthetic peptide
WGGDGFYAMDY

SEQ ID NO: 294 - protein, 108 aa, synthetic construct
  REGION 1..108: note = Description of Artificial Sequence: Synthetic polypeptide
DIVMTQSHKFMSTSVGDRVSITCKASQDVNTAVAWYQQKPGHSPKLLIYSASFRYTGVPDRFTGSRSGTDFTFTISSVQAEDLAVYYCQQHYTTPPTFGGGTKVEIKR

SEQ ID NO: 295 - protein, 8 aa, synthetic construct
  REGION 1..8: note = Description of Artificial Sequence: Synthetic peptide
QDVNTAVA

SEQ ID NO: 296 - protein, 7 aa, synthetic construct
  REGION 1..7: note = Description of Artificial Sequence: Synthetic peptide
SASFRYT

SEQ ID NO: 297 - protein, 9 aa, synthetic construct
  REGION 1..9: note = Description of Artificial Sequence: Synthetic peptide
QQHYTTPPT

SEQ ID NO: 298 - protein, 1255 aa, Homo sapiens [sequence omitted]

SEQ ID NO: 299 - protein, 449 aa, synthetic construct
  REGION 1..449: note = Description of Artificial Sequence: Synthetic polypeptide
EVQLVESGGGLVQPGGSLRLSCAASGFNIKDTYIHWVRQAPGKGLEWVARIYPTNGYTRYADSVKGRFTISADTSKNTAYLQMNSLRAEDTAVYYCSRWGGDGFYAMDYWGQGTLVTVSSASTKGPSVFPLAPSSKSTSGGTAALGCLVKDYFPEPVTVSWNSGALTSGVHTFPAVLQSSGLYSLSSVVTVPSSSLGTQTYICNVNHKPSNTKVDKKVEPKSCDKTHTCPPCPAPELLGGPSVFLFPPKPKDTLMISRTPEVTCVVVDVSHEDPEVKFNWYVDGVEVHNAKTKPREEQYNSTYRVVSVLTVLHQDWLNGKEYKCKVSNKALPAPIEKTISKAKGQPREPQVCTLPPSRDELTENQVSLTCLVKGFYPSDIAVEWESNGQPENNYKTTPPVLDSDGSFFLYSWLTVDKSRWQQGNVFSCSVMHEALHNHYTQKSLSLSPG

SEQ ID NO: 300 - protein, 449 aa, synthetic construct
  REGION 1..449: note = Description of Artificial Sequence: Synthetic polypeptide
EVQLVESGGGLVQPGGSLRLSCAASGFNIKDTYIHWVRQAPGKGLEWVARIYPTNGYTRYADSVKGRFTISADTSKNTAYLQMNSLRAEDTAVYYCSRWGGDGFYAMDYWGQGTLVTVSSASTKGPSVFPLAPSSKSTSGGTAALGCLVKDYFPEPVTVSWNSGALTSGVHTFPAVLQSSGLYSLSSVVTVPSSSLGTQTYICNVNHKPSNTKVDKKVEPKSCDKTHTCPPCPAPELLGGPSVFLFPPKPKDTLMISRTPEVTCVVVDVSHEDPEVKFNWYVDGVEVHNAKTKPREEQYNSTYRVVSVLTVLHQDWLNGKEYKCKVSNKALPAPIEKTISKAKGQPREPRVYTLPPCRDELTKNQVSLTCLVKGFYPSDIAVEWESNGQPENNYKTTPPVLVSDGSFTLYSKLTVDKSRWQQGNVFSCSVMHEALHNHYTQKSLSLSPG

SEQ ID NO: 301 - protein, 449 aa, synthetic construct
  REGION 1..449: note = Description of Artificial Sequence: Synthetic polypeptide
EVQLVESGGGLVQPGGSLRLSCAASGFNIKDTYIHWVRQAPGKGLEWVARIYPTNGYTRYADSVKGRFTISADTSKNTAYLQMNSLRAEDTAVYYCSRWGGDGFYAMDYWGQGTLVTVSSASTKGPSVFPLAPSSKSTSGGTAALGCLVKDYFPEPVTVSWNSGALTSGVHTFPAVLQSSGLYSLSSVVTVPSSSLGTQTYICNVNHKPSNTKVDKKVEPKSCDKTHTCPPCPAPELLGGPSVFLFPPKPKDTLMISRTPEVTCVVVDVSHEDPEVKFNWYVDGVEVHNAKTKPREEQYNSTYRVVSVLTVLHQDWLNGKEYKCKVSNKALPAPIEKTISKAKGQPREPQVYTLPPCRDELTKNQVSLWCLVKGFYPSDIAVEWESNGQPENNYKTTPPVLDSDGSFFLYSKLTVDKSRWQQGNVFSCSVMHEALHNHYTQKSLSLSPG

SEQ ID NO: 302 - protein, 449 aa, synthetic construct
  REGION 1..449: note = Description of Artificial Sequence: Synthetic polypeptide
EVQLVESGGGLVQPGGSLRLSCAASGFNIKDTYIHWVRQAPGKGLEWVARIYPTNGYTRYADSVKGRFTISADTSKNTAYLQMNSLRAEDTAVYYCSRWGGDGFYAMDYWGQGTLVTVSSASTKGPSVFPLAPSSKSTSGGTAALGCLVKDYFPEPVTVSWNSGALTSGVHTFPAVLQSSGLYSLSSVVTVPSSSLGTQTYICNVNHKPSNTKVDKKVEPKSCDKTHTCPPCPAPELLGGPSVFLFPPKPKDTLMISRTPEVTCVVVDVSHEDPEVKFNWYVDGVEVHNAKTKPREEQYNSTYRVVSVLTVLHQDWLNGKEYKCKVSNKALPAPIEKTISKAKGQPREPQVCTLPPSRDELTKNQVSLSCAVKGFYPSDIAVEWESNGQPENNYKTTPPVLDSDGSFFLVSKLTVDKSRWQQGNVFSCSVMHEALHNHYTQKSLSLSPG

SEQ ID NO: 303 - protein, 475 aa, synthetic construct
  REGION 1..475: note = Description of Artificial Sequence: Synthetic polypeptide
DIQMTQSPSSLSASVGDRVTITCRASQDVNTAVAWYQQKPGKAPKLLIYSASFLYSGVPSRFSGSRSGTDFTLTISSLQPEDFATYYCQQHYTTPPTFGCGTKVEIKGGGGSGGGGSGGGGSGGGGSEVQLVESGGGLVQPGGSLRLSCAASGFNIKDTYIHWVRQAPGKCLEWVARIYPTNGYTRYADSVKGRFTISADTSKNTAYLQMNSLRAEDTAVYYCSRWGGDGFYAMDYWGQGTLVTVSSASDKTHTCPPCPAPELLGGPSVFLFPPKPKDTLMISRTPEVTCVVVDVSHEDPEVKFNWYVDGVEVHNAKTKPREEQYNSTYRVVSVLTVLHQDWLNGKEYKCKVSNKALPAPIEKTISKAKGQPREPQVYTLPPCRDELTKNQVSLWCLVKGFYPSDIAVEWESNGQPENNYKTTPPVLDSDGSFFLYSKLTVDKSRWQQGNVFSCSVMHEALHNHYTQKSLSLSPG

SEQ ID NO: 304 - protein, 475 aa, synthetic construct
  REGION 1..475: note = Description of Artificial Sequence: Synthetic polypeptide
DIQMTQSPSSLSASVGDRVTITCRASQDVNTAVAWYQQKPGKAPKLLIYSASFLYSGVPSRFSGSRSGTDFTLTISSLQPEDFATYYCQQHYTTPPTFGCGTKVEIKGGGGSGGGGSGGGGSGGGGSEVQLVESGGGLVQPGGSLRLSCAASGFNIKDTYIHWVRQAPGKCLEWVARIYPTNGYTRYADSVKGRFTISADTSKNTAYLQMNSLRAEDTAVYYCSRWGGDGFYAMDYWGQGTLVTVSSASDKTHTCPPCPAPELLGGPSVFLFPPKPKDTLMISRTPEVTCVVVDVSHEDPEVKFNWYVDGVEVHNAKTKPREEQYNSTYRVVSVLTVLHQDWLNGKEYKCKVSNKALPAPIEKTISKAKGQPREPQVCTLPPSRDELTKNQVSLSCAVKGFYPSDIAVEWESNGQPENNYKTTPPVLDSDGSFFLVSKLTVDKSRWQQGNVFSCSVMHEALHNHYTQKSLSLSPG

SEQ ID NO: 305 - protein, 475 aa, synthetic construct
  REGION 1..475: note = Description of Artificial Sequence: Synthetic polypeptide
DIQMTQSPSSLSASVGDRVTITCRASQDVNTAVAWYQQKPGKAPKLLIYSASFLYSGVPSRFSGSRSGTDFTLTISSLQPEDFATYYCQQHYTTPPTFGCGTKVEIKGGGGSGGGGSGGGGSGGGGSEVQLVESGGGLVQPGGSLRLSCAASGFNIKDTYIHWVRQAPGKCLEWVARIYPTNGYTRYADSVKGRFTISADTSKNTAYLQMNSLRAEDTAVYYCSRWGGDGFYAMDYWGQGTLVTVSSASDKTHTCPPCPAPELLGGPSVFLFPPKPKDTLMISRTPEVTCVVVDVSHEDPEVKFNWYVDGVEVHNAKTKPREEQYNSTYRVVSVLTVLHQDWLNGKEYKCKVSNKALPAPIEKTISKAKGQPREPQVCTLPPSRDELTENQVSLTCLVKGFYPSDIAVEWESNGQPENNYKTTPPVLDSDGSFFLYSWLTVDKSRWQQGNVFSCSVMHEALHNHYTQKSLSLSPG

SEQ ID NO: 306 - protein, 475 aa, synthetic construct
  REGION 1..475: note = Description of Artificial Sequence: Synthetic polypeptide
DIQMTQSPSSLSASVGDRVTITCRASQDVNTAVAWYQQKPGKAPKLLIYSASFLYSGVPSRFSGSRSGTDFTLTISSLQPEDFATYYCQQHYTTPPTFGCGTKVEIKGGGGSGGGGSGGGGSGGGGSEVQLVESGGGLVQPGGSLRLSCAASGFNIKDTYIHWVRQAPGKCLEWVARIYPTNGYTRYADSVKGRFTISADTSKNTAYLQMNSLRAEDTAVYYCSRWGGDGFYAMDYWGQGTLVTVSSASDKTHTCPPCPAPELLGGPSVFLFPPKPKDTLMISRTPEVTCVVVDVSHEDPEVKFNWYVDGVEVHNAKTKPREEQYNSTYRVVSVLTVLHQDWLNGKEYKCKVSNKALPAPIEKTISKAKGQPREPRVYTLPPCRDELTKNQVSLTCLVKGFYPSDIAVEWESNGQPENNYKTTPPVLVSDGSFTLYSKLTVDKSRWQQGNVFSCSVMHEALHNHYTQKSLSLSPG

SEQ ID NO: 307 - protein, 5 aa, synthetic construct
  REGION 1..5: note = Description of Artificial Sequence: Synthetic peptide
GYYWS

SEQ ID NO: 308 - protein, 9 aa, synthetic construct
  REGION 1..9: note = Description of Artificial Sequence: Synthetic peptide
ARGPWSFDP

SEQ ID NO: 309 - protein, 5 aa, synthetic construct
  REGION 1..5: note = Description of Artificial Sequence: Synthetic peptide
SYAIS

SEQ ID NO: 310 - protein, 16 aa, synthetic construct
  REGION 1..16: note = Description of Artificial Sequence: Synthetic peptide
GDSSIRHAYYYYGMDV

SEQ ID NO: 311 - protein, 7 aa, synthetic construct
  REGION 1..7: note = Description of Artificial Sequence: Synthetic peptide
SSSYYWG

SEQ ID NO: 312 - protein, 11 aa, synthetic construct
  REGION 1..11: note = Description of Artificial Sequence: Synthetic peptide
GSDRFHPYFDY

SEQ ID NO: 313 - protein, 5 aa, synthetic construct
  REGION 1..5: note = Description of Artificial Sequence: Synthetic peptide
SYYMH

SEQ ID NO: 314 - protein, 17 aa, synthetic construct
  REGION 1..17: note = Description of Artificial Sequence: Synthetic peptide
GAPNYGDTTHDYYYMDV

SEQ ID NO: 315 - protein, 5 aa, synthetic construct
  REGION 1..5: note = Description of Artificial Sequence: Synthetic peptide
GYYMH

SEQ ID NO: 316 - protein, 15 aa, synthetic construct
  REGION 1..15: note = Description of Artificial Sequence: Synthetic peptide
DTGEYYDTDDHGMDV

SEQ ID NO: 317 - protein, 5 aa, synthetic construct
  REGION 1..5: note = Description of Artificial Sequence: Synthetic peptide
SYAMS

SEQ ID NO: 318 - protein, 12 aa, synthetic construct
  REGION 1..12: note = Description of Artificial Sequence: Synthetic peptide
DGGYYDSGAGDY

SEQ ID NO: 319 - protein, 5 aa, synthetic construct
  REGION 1..5: note = Description of Artificial Sequence: Synthetic peptide
SYSMN

SEQ ID NO: 320 - protein, 13 aa, synthetic construct
  REGION 1..13: note = Description of Artificial Sequence: Synthetic peptide
GAPMGAAAGWFDP

SEQ ID NO: 321 - protein, 16 aa, synthetic construct
  REGION 1..16: note = Description of Artificial Sequence: Synthetic peptide
EGAGFAYGMDYYYMDV

SEQ ID NO: 322 - protein, 122 aa, synthetic construct
  REGION 1..122: note = Description of Artificial Sequence: Synthetic polypeptide
EVQLVESGGGLVKPGGSLRLSCAASGFTFSSYSMNWVRQAPGKGLEWVSSISSSSSYIYYADSVKGRFTISRDNAKNSLYLQMNSLRAEDTAVYYCARGAPIGAAAGWFDPWGQGTLVTVSS

SEQ ID NO: 323 - protein, 15 aa, synthetic construct
  REGION 1..15: note = Description of Artificial Sequence: Synthetic peptide
ARGAPIGAAAGWFDP

SEQ ID NO: 324 - protein, 13 aa, synthetic construct
  REGION 1..13: note = Description of Artificial Sequence: Synthetic peptide
GAPIGAAAGWFDP

SEQ ID NO: 325 - protein, 122 aa, synthetic construct
  REGION 1..122: note = Description of Artificial Sequence: Synthetic polypeptide
EVQLVESGGGLVKPGGSLRLSCAASGFTFSSYSMNWVRQAPGKGLEWVSSISSSSSYIYYADSVKGRFTISRDNAKNSLYLQMNSLRAEDTAVYYCARGAPQGAAAGWFDPWGQGTLVTVSS

SEQ ID NO: 326 - protein, 15 aa, synthetic construct
  REGION 1..15: note = Description of Artificial Sequence: Synthetic peptide
ARGAPQGAAAGWFDP

SEQ ID NO: 327 - protein, 13 aa, synthetic construct
  REGION 1..13: note = Description of Artificial Sequence: Synthetic peptide
GAPQGAAAGWFDP

SEQ ID NO: 328 - protein, 122 aa, synthetic construct
  REGION 1..122: note = Description of Artificial Sequence: Synthetic polypeptide
EVQLVESGGGLVKPGGSLRLSCAASGFTFSSYSMNWVRQAPGKGLEWVSSISSSSSYIYYADSVKGRFTISRDNAKNSLYLQMNSLRAEDTAVYYCARGAPLGAAAGWFDPWGQGTLVTVSS

SEQ ID NO: 329 - protein, 15 aa, synthetic construct
  REGION 1..15: note = Description of Artificial Sequence: Synthetic peptide
ARGAPLGAAAGWFDP

SEQ ID NO: 330 - protein, 13 aa, synthetic construct
  REGION 1..13: note = Description of Artificial Sequence: Synthetic peptide
GAPLGAAAGWFDP

SEQ ID NO: 331 - protein, 122 aa, synthetic construct
  REGION 1..122: note = Description of Artificial Sequence: Synthetic polypeptide
EVQLVESGGGLVKPGGSLRLSCAASGFTFSSYSMNWVRQAPGKGLEWVSSISSSSSYIYYADSVKGRFTISRDNAKNSLYLQMNSLRAEDTAVYYCARGAPFGAAAGWFDPWGQGTLVTVSS

SEQ ID NO: 332 - protein, 15 aa, synthetic construct
  REGION 1..15: note = Description of Artificial Sequence: Synthetic peptide
ARGAPFGAAAGWFDP

SEQ ID NO: 333 - protein, 13 aa, synthetic construct
  REGION 1..13: note = Description of Artificial Sequence: Synthetic peptide
GAPFGAAAGWFDP

SEQ ID NO: 334 - protein, 122 aa, synthetic construct
  REGION 1..122: note = Description of Artificial Sequence: Synthetic polypeptide
EVQLVESGGGLVKPGGSLRLSCAASGFTFSSYSMNWVRQAPGKGLEWVSSISSSSSYIYYADSVKGRFTISRDNAKNSLYLQMNSLRAEDTAVYYCARGAPVGAAAGWFDPWGQGTLVTVSS

SEQ ID NO: 335 - protein, 15 aa, synthetic construct
  REGION 1..15: note = Description of Artificial Sequence: Synthetic peptide
ARGAPVGAAAGWFDP

SEQ ID NO: 336 - protein, 13 aa, synthetic construct
  REGION 1..13: note = Description of Artificial Sequence: Synthetic peptide
GAPVGAAAGWFDP

SEQ ID NO: 337 - protein, 122 aa, synthetic construct
  REGION 1..122: note = Description of Artificial Sequence: Synthetic polypeptide
  VARIANT 102: note = X is Met, Leu, Ile, Val, Gln, or Phe
EVQLVESGGGLVKPGGSLRLSCAASGFTFSSYSMNWVRQAPGKGLEWVSSISSSSSYIYYADSVKGRFTISRDNAKNSLYLQMNSLRAEDTAVYYCARGAPXGAAAGWFDPWGQGTLVTVSS

SEQ ID NO: 338 - protein, 15 aa, synthetic construct
  REGION 1..15: note = Description of Artificial Sequence: Synthetic peptide
  VARIANT 6: note = X is Met, Leu, Ile, Val, Gln, or Phe
ARGAPXGAAAGWFDP

SEQ ID NO: 339 - protein, 13 aa, synthetic construct
  REGION 1..13: note = Description of Artificial Sequence: Synthetic peptide
  VARIANT 4: note = X is Met, Leu, Ile, Val, Gln, or Phe
GAPXGAAAGWFDP

SEQ ID NO: 340 - protein, 9 aa, Homo sapiens
ILAKFLHWL

SEQ ID NO: 341 - protein, 9 aa, Homo sapiens
KIFGSLAFL

SEQ ID NO: 342 - protein, 9 aa, Homo sapiens
RMFPNAPYL

SEQ ID NO: 343 - protein, 13 aa, Homo sapiens
CASSFNMATGQYF

SEQ ID NO: 344 - protein, 10 aa, Homo sapiens
EAAGIGILTV

SEQ ID NO: 345 - protein, 9 aa, Homo sapiens
KASEKIFYV

SEQ ID NO: 346 - protein, 10 aa, Homo sapiens
ELTLGEFLKL

SEQ ID NO: 347 - protein, 9 aa, Homo sapiens
QLLALLPSL

SEQ ID NO: 348 - protein, 9 aa, Homo sapiens
SLLMWITQC

SEQ ID NO: 349 - protein, 200 aa, synthetic construct
  REGION 1..200: note = Description of Artificial Sequence: Synthetic polypeptide
KEVEQNSGPLSVPEGAIASLNCTYSDRGSQSFFWYRQYSGKSPELIMSIYSNGDKEDGRFTAQLNKASQYVSLLIRDSQPSDSATYLCAVTTDSWGKLQFGAGTQVVVTPDIQNPDPAVYQLRDSKSSDKSVCLFTDFDSQTNVSQSKDSDVYITDKTVLDMRSMDFKSNSAVAWSNKSDFACANAFNNSIIPEDTFFPS

SEQ ID NO: 350 - protein, 245 aa, synthetic construct
  REGION 1..245: note = Description of Artificial Sequence: Synthetic polypeptide
NAGVTQTPKFQVLKTGQSMTLQCAQDMNHEYMSWYRQDPGMGLRLIHYSVGAGITDQGEVPNGYNVSRSTTEDFPLRLLSAAPSQTSVYFCASRPGLAGGRPEQYFGPGTRLTVTEDLKNVFPPEVAVFEPSEAEISHTQKATLVCLATGFYPDHVELSWWVNGKEVHSGVSTDPQPLKEQPALNDSRYALSSRLRVSATFWQDPRNHFRCQVQFYGLSENDEWTQDRAKPVTQIVSAEAWGRAD

SEQ ID NO: 351 - protein, 115 aa, synthetic construct
  REGION 1..115: note = Description of Artificial Sequence: Synthetic polypeptide
KEVEQNSGPLSVPEGAIASLNCTYSDRGSQSFFWYRQYSGKSPELIMSIYSNGDKEDGRFTAQLNKASQYVSLLIRDSQPSDSATYLCAVTTDSWGKLQFGAGTQVVVTPDIQNP

SEQ ID NO: 352 - protein, 122 aa, synthetic construct
  REGION 1..122: note = Description of Artificial Sequence: Synthetic polypeptide
NAGVTQTPKFQVLKTGQSMTLQCAQDMNHEYMSWYRQDPGMGLRLIHYSVGAGITDQGEVPNGYNVSRSTTEDFPLRLLSAAPSQTSVYFCASRPGLAGGRPEQYFGPGTRLTVTEDLKNVF

SEQ ID NO: 353 - protein, 13 aa, synthetic construct
  REGION 1..13: note = Description of Artificial Sequence: Synthetic peptide
CAVTTDSWGKLQF

SEQ ID NO: 354 - protein, 16 aa, synthetic construct
  REGION 1..16: note = Description of Artificial Sequence: Synthetic peptide
CASRPGLAGGRPEQYF

SEQ ID NO: 355 - protein, 199 aa, synthetic construct
  REGION 1..199: note = Description of Artificial Sequence: Synthetic polypeptide
EVEQDPGPLSVPEGAIVSLNCTYSNSAFQYFMWYRQYSRKGPELLMYTYSSGNKEDGRFTAQVDKSSKYISLFIRDSQPSDSATYLCAMRGDSSYKLIFGSGTRLLVRPDIQNPDPAVYQLRDSKSSDKSVCLFTDFDSQTNVSQSKDSDVYITDKCVLDMRSMDFKSNSAVAWSNKSDFACANAFNNSIIPEDTFFPS

SEQ ID NO: 356 - protein, 245 aa, synthetic construct
  REGION 1..245: note = Description of Artificial Sequence: Synthetic polypeptide
AGVIQSPRHEVTEMGQQVTLRCKPISGHDYLFWYRQTMMRGLELLIYFNNNVPIDDSGMPEDRFSAKMPNASFSTLKIQPSEPRDSAVYFCASSLWEKLAKNIQYFGAGTRLSVLEDLKNVFPPEVAVFEPSEAEISHTQKATLVCLATGFYPDHVELSWWVNGKEVHSGVCTDPQPLKEQPALNDSRYALSSRLRVSATFWQDPRNHFRCQVQFYGLSENDEWTQDRAKPVTQIVSAEAWGRAD

SEQ ID NO: 357 - protein, 114 aa, synthetic construct
  REGION 1..114: note = Description of Artificial Sequence: Synthetic polypeptide
EVEQDPGPLSVPEGAIVSLNCTYSNSAFQYFMWYRQYSRKGPELLMYTYSSGNKEDGRFTAQVDKSSKYISLFIRDSQPSDSATYLCAMRGDSSYKLIFGSGTRLLVRPDIQNP

SEQ ID NO: 358 - protein, 122 aa, synthetic construct
  REGION 1..122: note = Description of Artificial Sequence: Synthetic polypeptide
AGVIQSPRHEVTEMGQQVTLRCKPISGHDYLFWYRQTMMRGLELLIYFNNNVPIDDSGMPEDRFSAKMPNASFSTLKIQPSEPRDSAVYFCASSLWEKLAKNIQYFGAGTRLSVLEDLKNVF

SEQ ID NO: 359 - protein, 13 aa, synthetic construct
  REGION 1..13: note = Description of Artificial Sequence: Synthetic peptide
CAMRGDSSYKLIF

SEQ ID NO: 360 - protein, 16 aa, synthetic construct
  REGION 1..16: note = Description of Artificial Sequence: Synthetic peptide
CASSLWEKLAKNIQYF

SEQ ID NO: 361 - protein, 200 aa, synthetic construct
  REGION 1..200: note = Description of Artificial Sequence: Synthetic polypeptide
IQVEQSPPDLILQEGANSTLRCNFSDSVNNLWWFHQNPWGQLINLFYIPSGTKQNGRLSATTVATERYSLLYISSSQTTDSGVYFCAVDSATALPYGYIFGTGTRLKVLANIQNPDPAVYQLRDSKSSDKSVCLFTDFDSQTNVSQSKDSDVYITDKCVLDMRSMDFKSNSAVAWSNKSDFACANAFNNSIIPEDTFFPS

SEQ ID NO: 362 - protein, 240 aa, synthetic construct
  REGION 1..240: note = Description of Artificial Sequence: Synthetic polypeptide
AGVTQTPKFQVLKTGQSMTLQCAQDMNHEYMSWYRQDPGMGLRLIHYSIHPEYTDQGEVPNGYNVSRSTTEDFPLRLLSAAPSQTSVYFCASSYQGTEAFFGQGTRLTVVEDLNKVFPPEVAVFEPSEAEISHTQKATLVCLATGFYPDHVELSWWVNGKEVHSGVCTDPQPLKEQPALNDSRYALSSRLRVSATFWQDPRNHFRCQVQFYGLSENDEWTQDRAKPVTQIVSAEAWGRAD

SEQ ID NO: 363 - protein, 115 aa, synthetic construct
  REGION 1..115: note = Description of Artificial Sequence: Synthetic polypeptide
IQVEQSPPDLILQEGANSTLRCNFSDSVNNLWWFHQNPWGQLINLFYIPSGTKQNGRLSATTVATERYSLLYISSSQTTDSGVYFCAVDSATALPYGYIFGTGTRLKVLANIQNP

SEQ ID NO: 364 - protein, 117 aa, synthetic construct
  REGION 1..117: note = Description of Artificial Sequence: Synthetic polypeptide
AGVTQTPKFQVLKTGQSMTLQCAQDMNHEYMSWYRQDPGMGLRLIHYSIHPEYTDQGEVPNGYNVSRSTTEDFPLRLLSAAPSQTSVYFCASSYQGTEAFFGQGTRLTVVEDLNKVF

SEQ ID NO: 365 - protein, 15 aa, synthetic construct
  REGION 1..15: note = Description of Artificial Sequence: Synthetic peptide
CAVDSATALPYGYIF

SEQ ID NO: 366 - protein, 12 aa, synthetic construct
  REGION 1..12: note = Description of Artificial Sequence: Synthetic peptide
CASSYQGTEAFF

SEQ ID NO: 367 - protein, 16 aa, synthetic construct
  REGION 1..16: note = Description of Artificial Sequence: Synthetic peptide
CAMSLYYGGSQGNLIF

SEQ ID NO: 368 - protein, 19 aa, synthetic construct
  REGION 1..19: note = Description of Artificial Sequence: Synthetic peptide
CASSLEIFGGIADTDTQYF

SEQ ID NO: 369 - protein, 15 aa, synthetic construct
  REGION 1..15: note = Description of Artificial Sequence: Synthetic peptide
CAVNDQGGGADGLTF

SEQ ID NO: 370 - protein, 13 aa, synthetic construct
  REGION 1..13: note = Description of Artificial Sequence: Synthetic peptide
CASSWWDTGELFF

SEQ ID NO: 371 - protein, 13 aa, synthetic construct
  REGION 1..13: note = Description of Artificial Sequence: Synthetic peptide
CAVSEGGDYKLSF

SEQ ID NO: 372 - protein, 12 aa, synthetic construct
  REGION 1..12: note = Description of Artificial Sequence: Synthetic peptide
CAWGTLATEQYF

SEQ ID NO: 373 - protein, 197 aa, synthetic construct
  REGION 1..197: note = Description of Artificial Sequence: Synthetic polypeptide
AQEVTQIPAALSVPEGENLVLNCSFTDSAIYNLQWFRQDPGKGLTSLLYVRPYQREQTSGRLNASLDKSSGRSTLYIAASQPGDSATYLCAVRPGGAGPFFVVFGKGTKLSVIPNIQNPDPAVYQLRDSKSSDKSVCLFTDFDSQTNVSQSKDSDVYITDKCVLDMRSMDFKSNSAVAWSNKSDFACANAFNNSIIP

SEQ ID NO: 374 - protein, 241 aa, synthetic construct
  REGION 1..241: note = Description of Artificial Sequence: Synthetic polypeptide
AGVTQTPRYLIKTRGQQVTLSCSPISGHRSVSWYQQTPGQGLQFLFEYFSETQRNKGNFPGRFSGRQFSNSRSEMNVSTLELGDSALYLCASSFNMATGQYFGPGTRLTVTEDLKNVFPPEVAVFEPSEAEISHTQKATLVCLATGFYPDHVELSWWVNGKEVHSGVCTDPQPLKEQPALNDSRYALSSRLRVSATFWQDPRNHFRCQVQFYGLSENDEWTQDRAKPVTQIVSAEAWGRAD

SEQ ID NO: 375 - protein, 119 aa, synthetic construct
  REGION 1..119: note = Description of Artificial Sequence: Synthetic polypeptide
AQEVTQIPAALSVPEGENLVLNCSFTDSAIYNLQWFRQDPGKGLTSLLYVRPYQREQTSGRLNASLDKSSGRSTLYIAASQPGDSATYLCAVRPGGAGPFFVVFGKGTKLSVIPNIQNP

SEQ ID NO: 376 - protein, 118 aa, synthetic construct
  REGION 1..118: note = Description of Artificial Sequence: Synthetic polypeptide
AGVTQTPRYLIKTRGQQVTLSCSPISGHRSVSWYQQTPGQGLQFLFEYFSETQRNKGNFPGRFSGRQFSNSRSEMNVSTLELGDSALYLCASSFNMATGQYFGPGTRLTVTEDLKNVF

SEQ ID NO: 377 - protein, 12 aa, synthetic construct
  REGION 1..12: note = Description of Artificial Sequence: Synthetic peptide
CAVRPGGAGPFF

SEQ ID NO: 378 - protein, 13 aa, synthetic construct
  REGION 1..13: note = Description of Artificial Sequence: Synthetic peptide
CASSFNMATGQYF

SEQ ID NO: 379 - protein, 199 aa, synthetic construct
  REGION 1..199: note = Description of Artificial Sequence: Synthetic polypeptide
EVEQDPGPLSVPEGAIVSLNCTYSNSAFQYFMWYRQYSRKGPELLMYTYSSGNKEDGRFTAQVDKSSKYISLFIRDSQPSDSATYLCAMSETGGFKTIFGAGTRLFVKANIQNPDPAVYQLRDSKSSDKSVCLFTDFDSQTNVSQSKDSDVYITDKTVLDMRSMDFKSNSAVAWSNKSDFACANAFNNSIIPEDTFFPS

SEQ ID NO: 380 - protein, 244 aa, synthetic construct
  REGION 1..244: note = Description of Artificial Sequence: Synthetic polypeptide
EAQVTQNPRYLITVTGKKLTVTCSQNMNHEYMSWYRQDPGLGLRQIYYSMNVEVTDKGDVPEGYKVSRKEKRNFPLILESPSPNQTSLYFCASSLVGTAGSPLHFGNGTRLTVTEDLNKVFPPEVAVFEPSEAEISHTQKATLVCLATGFFPDHVELSWWVNGKEVHSGVSTDPQPLKEQPALNDSRYCLSSRLRVSATFWQNPRNHFRCQVQFYGLSENDEWTQDRAKPVTQIVSAEAWGRAD

SEQ ID NO: 381 - protein, 114 aa, synthetic construct
  REGION 1..114: note = Description of Artificial Sequence: Synthetic polypeptide
EVEQDPGPLSVPEGAIVSLNCTYSNSAFQYFMWYRQYSRKGPELLMYTYSSGNKEDGRFTAQVDKSSKYISLFIRDSQPSDSATYLCAMSETGGFKTIFGAGTRLFVKANIQNP

SEQ ID NO: 382 - protein, 121 aa, synthetic construct
  REGION 1..121: note = Description of Artificial Sequence: Synthetic polypeptide
EAQVTQNPRYLITVTGKKLTVTCSQNMNHEYMSWYRQDPGLGLRQIYYSMNVEVTDKGDVPEGYKVSRKEKRNFPLILESPSPNQTSLYFCASSLVGTAGSPLHFGNGTRLTVTEDLNKVF

SEQ ID NO: 383 - protein, 13 aa, synthetic construct
  REGION 1..13: note = Description of Artificial Sequence: Synthetic peptide
CAMSETGGFKTIF

SEQ ID NO: 384 - protein, 15 aa, synthetic construct
  REGION 1..15: note = Description of Artificial Sequence: Synthetic peptide
CASSLVGTAGSPLHF

SEQ ID NO: 385 - protein, 200 aa, synthetic construct
  REGION 1..200: note = Description of Artificial Sequence: Synthetic polypeptide
AQKITQTQPGMFVQEKEAVTLDCTYDTSDQSYGLFWYKQPSSGEMIFLIYQGSYDEQNATEGRYSLNFQKARKSANLVISASQLGDSAMYFCAMREGGGYNKLIFGAGTRLAVHPDPAVYQLRDSKSSDKSVCLFTDFDSQTNVSQSKDSDVYITDKTVLDMRSMDFKSNSAVAWSNKSDFACANAFNNSIIPEDTFFPS

SEQ ID NO: 386 - protein, 241 aa, synthetic construct
  REGION 1..241: note = Description of Artificial Sequence: Synthetic polypeptide
SQTIHQWPATLVQPVGSPLSLECTVEGTSNPNLYWYRQAAGRGLQLLFYSVGIGQISSEVPQNLSASRPQDRQFILSSKKLLLSDSGFYLCAGQDLNTEAFFGQGTRLTVVEDLNKVFPPEVAVFEPSEAEISHTQKATLVCLATGFYPDHVELSWWVNGKEVHSGVCTDPQPLKEQPALNDSRYALSSRLRVSATFWQDPRNHFRCQVQFYGLSENDEWTQDRAKPVTQIVSAEAWGRAD

SEQ ID NO: 387 - protein, 14 aa, synthetic construct
  REGION 1..14: note = Description of Artificial Sequence: Synthetic peptide
CAMTSGFGNEKLTF

SEQ ID NO: 388 - protein, 14 aa, synthetic construct
  REGION 1..14: note = Description of Artificial Sequence: Synthetic peptide
CATSRGQGGQPQHF

SEQ ID NO: 389 - protein, 14 aa, synthetic construct
  REGION 1..14: note = Description of Artificial Sequence: Synthetic peptide
CAETVTDSWGKLQF

SEQ ID NO: 390 - protein, 15 aa, synthetic construct
  REGION 1..15: note = Description of Artificial Sequence: Synthetic peptide
CATSRGDSTAEPQHF

SEQ ID NO: 391 - protein, 14 aa, synthetic construct
  REGION 1..14: note = Description of Artificial Sequence: Synthetic peptide
CAMREGGGYNKLIF

SEQ ID NO: 392 - protein, 12 aa, synthetic construct
  REGION 1..12: note = Description of Artificial Sequence: Synthetic peptide
CAGQDLNTEAFF

SEQ ID NO: 393 - protein, 204 aa, synthetic construct
  REGION 1..204: note = Description of Artificial Sequence: Synthetic polypeptide
AQSVTQLGSHVSVSERALVLLRCNYSSSVPPYLFWYVQYPNQGLQLLLKYTSAATLVKGINGFEAEFKKSETSFHLTKPSAHMSDAAEYFCAVSGQTGANNLFFGTGTRLTVIPYIQNPDPAVYQLRDSKSSDKSVCLFTDFDSQTNVSQSKDSDVYITDKTVLDMRSMDFKSNSAVAWSNKSDFACANAFNNSIIPEDTFFPS

SEQ ID NO: 394 - protein, 243 aa, synthetic construct
  REGION 1..243: note = Description of Artificial Sequence: Synthetic polypeptide
DSGVTQTPKHLITATGQRVTLRCSPRSGDLSVYWYQQSLDQGLQFLIQYYNGEERAKGNILERFSAQQFPDLHSELNLSSLELGDSALYFCASARWDRGGEQYFGPGTRLTVTEDLKNVFPPEVAVFEPSEAEISHTQKATLVCLATGFYPDHVELSWWVNGKEVHSGVSTDPQPLKEQPALNDSRYCLSSRLRVSATFWQNPRNHFRCQVQFYGLSENDEWTQDRAKPVTQIVSAEAWGRAD

SEQ ID NO: 395 - protein, 119 aa, synthetic construct
  REGION 1..119: note = Description of Artificial Sequence: Synthetic polypeptide
AQSVTQLGSHVSVSERALVLLRCNYSSSVPPYLFWYVQYPNQGLQLLLKYTSAATLVKGINGFEAEFKKSETSFHLTKPSAHMSDAAEYFCAVSGQTGANNLFFGTGTRLTVIPYIQNP

SEQ ID NO: 396 - protein, 120 aa, synthetic construct
  REGION 1..120: note = Description of Artificial Sequence: Synthetic polypeptide
DSGVTQTPKHLITATGQRVTLRCSPRSGDLSVYWYQQSLDQGLQFLIQYYNGEERAKGNILERFSAQQFPDLHSELNLSSLELGDSALYFCASARWDRGGEQYFGPGTRLTVTEDLKNVF

SEQ ID NO: 397 - protein, 13 aa, synthetic construct
  REGION 1..13: note = Description of Artificial Sequence: Synthetic peptide
CAVSGQTGANNLF

SEQ ID NO: 398 - protein, 14 aa, synthetic construct
  REGION 1..14: note = Description of Artificial Sequence: Synthetic peptide
CASARWDRGGEQYF

SEQ ID NO: 399 - protein, 203 aa, synthetic construct
  REGION 1..203: note = Description of Artificial Sequence: Synthetic polypeptide
GQQLNQSPQSMFIQEGEDVSMNCTSSSIFNTWLWYKQDPGEGPVLLIALYKAGELTSNGRLTAQFGITRKDSFLNISASIPSDVGIYFCAGIPRDNYGQNFVFGPGTRLSVLPYIQNPDPAVYQLRDSKSSDKSVCLFTDFDSQTNVSQSKDSDVYITDKTVLDMRSMDFKSNSAVAWSNKSDFACANAFNNSIIPEDTFFPS

SEQ ID NO: 400 - protein, 244 aa, synthetic construct
  REGION 1..244: note = Description of Artificial Sequence: Synthetic polypeptide
DVKVTQSSRYLVKRTGEKVFLECVQDMDHENMFWYRQDPGLGLRLIYFSYDVKMKEKGDIPEGYSVSREKKERFSLILESASTNQTSMYLCASTPWLAGGNEQFFGPGTRLTVLEDLKNVFPPEVAVFEPSEAEISHTQKATLVCLATGFYPDHVELSWWVNGKEVHSGVSTDPQPLKEQPALNDSRYCLSSRLRVSATFWQNPRNHFRCQVQFYGLSENDEWTQDRAKPVTQIVSAEAWGRAD

SEQ ID NO: 401 - protein, 118 aa, synthetic construct
  REGION 1..118: note = Description of Artificial Sequence: Synthetic polypeptide
GQQLNQSPQSMFIQEGEDVSMNCTSSSIFNTWLWYKQDPGEGPVLLIALYKAGELTSNGRLTAQFGITRKDSFLNISASIPSDVGIYFCAGIPRDNYGQNFVFGPGTRLSVLPYIQNP

SEQ ID NO: 402 - protein, 121 aa, synthetic construct
  REGION 1..121: note = Description of Artificial Sequence: Synthetic polypeptide
DVKVTQSSRYLVKRTGEKVFLECVQDMDHENMFWYRQDPGLGLRLIYFSYDVKMKEKGDIPEGYSVSREKKERFSLILESASTNQTSMYLCASTPWLAGGNEQFFGPGTRLTVLEDLKNVF

SEQ ID NO: 403 - protein, 15 aa, synthetic construct
  REGION 1..15: note = Description of Artificial Sequence: Synthetic peptide
CAGIPRDNYGQNFVF

SEQ ID NO: 404 - protein, 15 aa, synthetic construct
  REGION 1..15: note = Description of Artificial Sequence: Synthetic peptide
CASTPWLAGGNEQFF

SEQ ID NO: 405 - protein, 201 aa, synthetic construct
  REGION 1..201: note = Description of Artificial Sequence: Synthetic polypeptide
QKEVEQNSGPLSVPEGAIASLNCTYSDRGSQSFFWYRQYSGKSPELIMFIYSNGDKEDGRFTAQLNKASQYVSLLIRDSQPSDSATYLCAVKDNAGNMLTFGGGTRLMVKPHIQNPDPAVYQLRDSKSSDKSVCLFTDFDSQTNVSQSKDSDVYITDKTVLDMRSMDFKSNSAVAWSNKSDFACANAFNNSIIPEDTFFPS

SEQ ID NO: 406 - protein, 243 aa, synthetic construct
  REGION 1..243: note = Description of Artificial Sequence: Synthetic polypeptide
DSGVTQTPKHLITATGQRVTLRCSPRSGDLSVYWYQQSLDQGLQFLIQYYNGEERAKGNILERFSAQQFPDLHSELNLSSLELGDSALYFCASSDGGGVYEQYFGPGTRLTVTEDLKNVFPPEVAVFEPSEAEISHTQKATLVCLATGFYPDHVELSWWVNGKEVHSGVSTDPQPLKEQPALNDSRYCLSSRLRVSATFWQNPRNHFRCQVQFYGLSENDEWTQDRAKPVTQIVSAEAWGRAD

SEQ ID NO: 407 - protein, 116 aa, synthetic construct
  REGION 1..116: note = Description of Artificial Sequence: Synthetic polypeptide
QKEVEQNSGPLSVPEGAIASLNCTYSDRGSQSFFWYRQYSGKSPELIMFIYSNGDKEDGRFTAQLNKASQYVSLLIRDSQPSDSATYLCAVKDNAGNMLTFGGGTRLMVKPHIQNP

SEQ ID NO: 408 - protein, 120 aa, synthetic construct
  REGION 1..120: note = Description of Artificial Sequence: Synthetic polypeptide
DSGVTQTPKHLITATGQRVTLRCSPRSGDLSVYWYQQSLDQGLQFLIQYYNGEERAKGNILERFSAQQFPDLHSELNLSSLELGDSALYFCASSDGGGVYEQYFGPGTRLTVTEDLKNVF

SEQ ID NO: 409 - protein, 13 aa, synthetic construct
  REGION 1..13: note = Description of Artificial Sequence: Synthetic peptide
CAVKDNAGNMLTF

SEQ ID NO: 410 - protein, 14 aa, synthetic construct
  REGION 1..14: note = Description of Artificial Sequence: Synthetic peptide
CASSDGGGVYEQYF

SEQ ID NO: 411 - protein, 203 aa, synthetic construct [sequence omitted]

SEQ ID NO: 412 - protein, 241 aa, synthetic construct [sequence omitted]

SEQ ID NO: 413 - protein, 118 aa, synthetic construct
  REGION 1..118: note = Description of Artificial Sequence: Synthetic polypeptide
QEVTQIPAALSVPEGENLVLNCSFTDSAIYNLQWFRQDPGKGLTSLLLIQSSQREQTSGRLNASLDKSSGRSTLYIAASQPGDSATYLCAVRPTSGGSYIPTFGRGTSLIVHPYIQNP

SEQ ID NO: 414 - protein, 118 aa, synthetic construct
  REGION 1..118: note = Description of Artificial Sequence: Synthetic polypeptide
GVTQTPKFQVLKTGQSMTLQCAQDMNHEYMSWYRQDPGMGLRLIHYSVGAGITDQGEVPNGYNVSRSTTEDFPLRLLSAAPSQTSVYFCASSYVGNTGELFFGEGSRLTVLEDLKNVF

SEQ ID NO: 415 - protein, 15 aa, synthetic construct
  REGION 1..15: note = Description of Artificial Sequence: Synthetic peptide
CAVRPTSGGSYIPTF

SEQ ID NO: 416 - protein, 14 aa, synthetic construct
  REGION 1..14: note = Description of Artificial Sequence: Synthetic peptide
CASSYVGNTGELFF

SEQ ID NO: 417 - protein, 206 aa, synthetic construct
  REGION 1..206: note = Description of Artificial Sequence: Synthetic polypeptide
KQQVTQIPAALSVPEGENLVLNCSFTDSAIYNLQWFRQDPGGKLTSLLLIQSSQREQTSGRLNASLDKSAGSSTLYIAASQPGDSATYLCAVRPTSGGSYIPTFGRGTSLIVHPYIQNPDPAVYQLRDSKSSDKSVCLFTDFDSQTNVSQSKDSDVYITDKCVLDMRSMDFKSNSAVAWSNKSDFACANAFNNSIIPEDTFFPSPE

SEQ ID NO: 418 - protein, 119 aa, synthetic construct
  REGION 1..119: note = Description of Artificial Sequence: Synthetic polypeptide
KQQVTQIPAALSVPEGENLVLNCSFTDSAIYNLQWFRQDPGGKLTSLLLIQSSQREQTSGRLNASLDKSAGSSTLYIAASQPGDSATYLCAVRPTSGGSYIPTFGRGTSLIVHPYIQNP

SEQ ID NO: 419 - protein, 194 aa, synthetic construct
  REGION 1..194: note = Description of Artificial Sequence: Synthetic polypeptide
KQEVTQIPAALSVPEGENLVLNCSFTDSAIYNLQWFRQDPGKGLTSLLLIQSSQREQTSGRLNASLDKSSGSSTLYIAASQPGDSATYLCAVRPLLDGTYIPTFGRGTSLIVHPYIQNPDPAVYQLRDSKSSDKSVCLFTDFDSQTNVSQSKDSDVYITDKCVLDMRSMDFKSNSAVAWSNKSDFACANAFNNS

SEQ ID NO: 420 - protein, 241 aa, synthetic construct
  REGION 1..241: note = Description of Artificial Sequence: Synthetic polypeptide
GVTQTPKFQVLKTGQSMTLQCAQDMNHEYMSWYRQDPGMGLRLIHYSVGAGTTDQGEVPNGYNVSRSTIEDFPLRLLSAAPSQTSVYFCASSYLGNTGELFFGEGSRLTVLEDLKNVFPPEVAVFEPSEAEISHTQKATLVCLATGFYPDHVELSWWVNGKEVHSGVCTDPQPLKEQPALNDSRYALSSRLRVSATFWQDPRNHFRCQVQFYGLSENDEWTQDRAKPVTQIVSAEAWGRAD

SEQ ID NO: 421 - protein, 119 aa, synthetic construct
  REGION 1..119: note = Description of Artificial Sequence: Synthetic polypeptide
KQEVTQIPAALSVPEGENLVLNCSFTDSAIYNLQWFRQDPGKGLTSLLLIQSSQREQTSGRLNASLDKSSGSSTLYIAASQPGDSATYLCAVRPLLDGTYIPTFGRGTSLIVHPYIQNP

SEQ ID NO: 422 - protein, 118 aa, synthetic construct
  REGION 1..118: note = Description of Artificial Sequence: Synthetic polypeptide
GVTQTPKFQVLKTGQSMTLQCAQDMNHEYMSWYRQDPGMGLRLIHYSVGAGTTDQGEVPNGYNVSRSTIEDFPLRLLSAAPSQTSVYFCASSYLGNTGELFFGEGSRLTVLEDLKNVF

SEQ ID NO: 423 - protein, 15 aa, synthetic construct
  REGION 1..15: note = Description of Artificial Sequence: Synthetic peptide
CAVRPLLDGTYIPTF

SEQ ID NO: 424 - protein, 14 aa, synthetic construct
  REGION 1..14: note = Description of Artificial Sequence: Synthetic peptide
CASSYLGNTGELFF

SEQ ID NO: 425 - protein, 9 aa, Homo sapiens
LGYGFVNYI

SEQ ID NO: 426 - protein, 10 aa, Homo sapiens
ALWGPDPAAA

SEQ ID NO: 427 - protein, 20 aa, synthetic construct
  REGION 1..20: note = Description of Artificial Sequence: Synthetic peptide
GGGGSGGGGSGGGGSGGGGS

SEQ ID NO: 428 - protein, 197 aa, synthetic construct
  REGION 1..197: note = Description of Artificial Sequence: Synthetic polypeptide
EVEQDPGPLSVPEGAIVSLNCTYSNSAFQYFMWYRQYSRKGPELLMYTYSSGNKEDGRFTAQVDKSSKYISLFIRDSQPSDSATYLCAMSLYYGGSQGNLIFGKGTKLSVKPDPAVYQLRDSKSSDKSVCLFTDFDSQTNVSQSKDSDVYITDKCVLDMRSMDFKSNSAVAWSNKSDFACANAFNNSIIPEDTFFPS

SEQ ID NO: 429 - protein, 248 aa, synthetic construct
  REGION 1..248: note = Description of Artificial Sequence: Synthetic polypeptide
AGVAQSPRYKIIEKRQSVAFWCNPISGHATLYWYQQILGQGPKLLIQFQNNGVVDDSQLPKDRFSAERLKGVDSTLKIQPAKLEDSAVYLCASSLEIFGGIADTDTQYFGPGTRLTVLEDLKNVFPPEVAVFEPSEAEISHTQKATLVCLATGFYPDHVELSWWVNGKEVHSGVCTDPQPLKEQPALNDSRYALSSRLRVSATFWQDPRNHFRCQVQFYGLSENDEWTQDRAKPVTQIVSAEAWGRAD

SEQ ID NO: 430 - protein, 112 aa, synthetic construct
  REGION 1..112: note = Description of Artificial Sequence: Synthetic polypeptide
EVEQDPGPLSVPEGAIVSLNCTYSNSAFQYFMWYRQYSRKGPELLMYTYSSGNKEDGRFTAQVDKSSKYISLFIRDSQPSDSATYLCAMSLYYGGSQGNLIFGKGTKLSVKP

SEQ ID NO: 431 - protein, 125 aa, synthetic construct
  REGION 1..125: note = Description of Artificial Sequence: Synthetic polypeptide
AGVAQSPRYKIIEKRQSVAFWCNPISGHATLYWYQQILGQGPKLLIQFQNNGVVDDSQLPKDRFSAERLKGVDSTLKIQPAKLEDSAVYLCASSLEIFGGIADTDTQYFGPGTRLTVLEDLKNVF

SEQ ID NO: 432 - protein, 196 aa, synthetic construct
  REGION 1..196: note = Description of Artificial Sequence: Synthetic polypeptide
EVEQNSGPLSVPEGAIASLNCTYSDRGSQSFFWYRQYSGKSPELIMFIYSNGDKEDGRFTAQLNKASQYVSLLIRDSQPSDSATYLCAVNDQGGGADGLTFGKGTHLIIQPDPAVYQLRDSKSSDKSVCLFTDFDSQTNVSQSKDSDVYITDKCVLDMRSMDFKSNSAVAWSNKSDFACANAFNNSIIPEDTFFPS

SEQ ID NO: 433 - protein, 242 aa, synthetic construct
  REGION 1..242: note = Description of Artificial Sequence: Synthetic polypeptide
NAGVTQTPKFRVLKTGQSMTLLCAQDMNHEYMYWYRQDPGMGLRLIHYSVGEGTTAKGEVPDGYNVSRLKKQNFLLGLESAAPSQTSVYFCASSWWDTGELFFGEGSRLTVLEDLKNVFPPEVAVFEPSEAEISHTQKATLVCLATGFYPDHVELSWWVNGKEVHSGVCTDPQPLKEQPALNDSRYALSSRLRVSATFWQDPRNHFRCQVQFYGLSENDEWTQDRAKPVTQIVSAEAWGRAD

SEQ ID NO: 434 - protein, 111 aa, synthetic construct
  REGION 1..111: note = Description of Artificial Sequence: Synthetic polypeptide
EVEQNSGPLSVPEGAIASLNCTYSDRGSQSFFWYRQYSGKSPELIMFIYSNGDKEDGRFTAQLNKASQYVSLLIRDSQPSDSATYLCAVNDQGGGADGLTFGKGTHLIIQP

SEQ ID NO: 435 - protein, 119 aa, synthetic construct
  REGION 1..119: note = Description of Artificial Sequence: Synthetic polypeptide
NAGVTQTPKFRVLKTGQSMTLLCAQDMNHEYMYWYRQDPGMGLRLIHYSVGEGTTAKGEVPDGYNVSRLKKQNFLLGLESAAPSQTSVYFCASSWWDTGELFFGEGSRLTVLEDLKNVF

SEQ ID NO: 436 - protein, 197 aa, synthetic construct
  REGION 1..197: note = Description of Artificial Sequence: Synthetic polypeptide
AQSVTQLGSHVSVSEGALVLLRCNYSSSVPPYLFWYVQYPQGLQLLLKYTSAATLVKGINGFEAEFKKSETSFHLTKPSAHMSDAAEYFCAVSEGGDYKLSFGAGTTVTVRADPAVYQLRDSKSSDKSVCLFTDFDSQTNVSQSKDSDVYITDKCVLDMRSMDFKSNSAVAWSNKSDFACANAFNNSIIPEDTFFPS

SEQ ID NO: 437 - protein, 241 aa, synthetic construct
  REGION 1..241: note = Description of Artificial Sequence: Synthetic polypeptide
DVKVTQSSRYLVKRTGEKVFLECVQDMDHENMFWYRQDPGLGLRLIYFSYDVKMKEKGDIPEGYSVSREKKERFSLILESASTNQTSMYLCAWGTLATEQYFGPGTRLTVTEDLKNVFPPEVAVFEPSEAEISHTQKATLVCLATGFYPDHVELSWWVNGKEVHSGVCTDPQPLKEQPALNDSRYALSSRLRVSATFWQDPRNHFRCQVQFYGLSENDEWTQDRAKPVTQIVSAEAWGRAD

SEQ ID NO: 438 - protein, 112 aa, synthetic construct
  REGION 1..112: note = Description of Artificial Sequence: Synthetic polypeptide
AQSVTQLGSHVSVSEGALVLLRCNYSSSVPPYLFWYVQYPQGLQLLLKYTSAATLVKGINGFEAEFKKSETSFHLTKPSAHMSDAAEYFCAVSEGGDYKLSFGAGTTVTVRA

SEQ ID NO: 439 - protein, 118 aa, synthetic construct
  REGION 1..118: note = Description of Artificial Sequence: Synthetic polypeptide
DVKVTQSSRYLVKRTGEKVFLECVQDMDHENMFWYRQDPGLGLRLIYFSYDVKMKEKGDIPEGYSVSREKKERFSLILESASTNQTSMYLCAWGTLATEQYFGPGTRLTVTEDLKNVF

SEQ ID NO: 440 - protein, 101 aa, synthetic construct
  REGION 1..101: note = Description of Artificial Sequence: Synthetic polypeptide
WGKLQFGAGTQVVVTPDPAVYQLRDSKSSDKSVCLFTDFDSQTNVSQSKDSDVYITDKTVLDMRSMDFKSNSAVAWSNKSDFACANAFNNSIIPEDTFFPS

SEQ ID NO: 441 - protein, 133 aa, synthetic construct
  REGION 1..133: note = Description of Artificial Sequence: Synthetic polypeptide
SILEDLNKVFPPEVAVFEPSEAEISHTQKATLVCLATGFYPDHVELSWWVNGKEVHSGVCTDPQPLKEQPALNDSRYALSSRLRVSATFWQDPRNHFRCQVQFYGLSENDEWTQDRAKPVTQIVSAEAWGRAD

SEQ ID NO: 442 - protein, 117 aa, synthetic construct
  REGION 1..117: note = Description of Artificial Sequence: Synthetic polypeptide
GESVGLHLPTLSVQEGDNSIINCAYSNSASDYFIWYKQESGKGPQFIIDIRSNMDKRQGQRVTVLLNKTVKHLSLQIAATQPGDSAVYFCAENCAETVTDSWGKLQFGAGTQVVVTP

SEQ ID NO: 443 - protein, 121 aa, synthetic construct
  REGION 1..121: note = Description of Artificial Sequence: Synthetic polypeptide
DAMVIQNPRYQVTQFGKPVTLSCSQTLNHNVMYWYQQKSSQAPKLLFHYYDKDFNNEADTPDNFQSRRPNTSFCFLDIRSPGLGDAAMYLCATSRGDSTAEPQHFGDGTRLSILEDLNKVF

SEQ ID NO: 444 - protein, 115 aa, synthetic construct
  REGION 1..115: note = Description of Artificial Sequence: Synthetic polypeptide
AQKITQTQPGMFVQEKEAVTLDCTYDTSDQSYGLFWYKQPSSGEMIFLIYQGSYDEQNATEGRYSLNFQKARKSANLVISASQLGDSAMYFCAMREGGGYNKLIFGAGTRLAVHP

SEQ ID NO: 445 - protein, 118 aa, synthetic construct
  REGION 1..118: note = Description of Artificial Sequence: Synthetic polypeptide
SQTIHQWPATLVQPVGSPLSLECTVEGTSNPNLYWYRQAAGRGLQLLFYSVGIGQISSEVPQNLSASRPQDRQFILSSKKLLLSDSGFYLCAGQDLNTEAFFGQGTRLTVVEDLNKVF